European Patent Specification EP 3 365 452 B1, published October 18, 2023. Title: Production of Proteins. Applicant: The University of Manchester. The sequence listing filed with the application follows.

SEQUENCE LISTING (48 sequences)

SEQ ID NO: 1 - protein, 17 aa, Artificial Sequence
  Gaussia luciferase signal peptide
MGVKVLFALICIAVAEA

SEQ ID NO: 2 - protein, 24 aa, Artificial Sequence
  PDX-Furin inhibitor signal peptide
MPSSVSWGILLLAGLCCLVPVSLA

SEQ ID NO: 3 - protein, 17 aa, Artificial Sequence
  BM40 signal peptide
MRAWIFFLLCLAGRALA

SEQ ID NO: 4 - DNA, 298 bp, Artificial Sequence
  DNA fragment 1
gctgggtaccgaaattaatacgactcactatagggagacccaagctggcttgcgtttaaacttaagcttagcgcagaggcttggggcagccgagcggcagccaggccccggcccgggcctcggttccagaagggagaggagcccgccaaggcgcgcaagagagcgggctgcctcgcagtccgagccggagagggagcgcgagccgcgccggccccggacggcctccgaaaccatgagggcctggatcttctttctcctttgcctggccgggagggctctggcagccccgctagccgag

SEQ ID NO: 5 - DNA, 301 bp, Artificial Sequence
  DNA fragment 2
gctgggtaccgaaattaatacgactcactatagggagacccaagctggcttgcgtttaaacttaagcttagcgcagaggcttggggcagccgagcggcagccaggccccggcccgggcctcggttccagaagggagaggagcccgccaaggcgcgcaagagagcgggctgcctcgcagtccgagccggagagggagcgcgagccgcgccggccccggacggcctccgaaaccatgggagtcaaagttctgtttgccctgatctgcatcgctgtggccgaggccaagcccacgctagccgag

SEQ ID NO: 6 - DNA, 116 bp, Artificial Sequence
  DNA fragment 3
gctgggtaccgaaattaatacgactcactataggggaaccagccaccatgggagtcaaagttctgtttgccctgatctgcatcgctgtggccgaggccaagcccacgctagccgag

SEQ ID NO: 7 - DNA, 428 bp, Artificial Sequence
  F1ori sequence
gcgccctgtagcggcgcattaagcgcggcgggtgtggtggttacgcgcagcgtgaccgctacacttgccagcgccctagcgcccgctcctttcgctttcttcccttcctttctcgccacgttcgccggctttccccgtcaagctctaaatcgggggctccctttagggttccgatttagtgctttacggcacctcgaccccaaaaaacttgattagggtgatggttcacgtagtgggccatcgccctgatagacggtttttcgccctttgacgttggagtccacgttctttaatagtggactcttgttccaaactggaacaacactcaaccctatctcggtctattcttttgatttataagggattttgccgatttcggcctattggttaaaaaatgagctgatttaacaaaaatttaacgcgaatta

SEQ ID NO: 8 - DNA, 74 bp, Artificial Sequence
  EM7 sequence
cagcacgtgttgacaattaatcatcggcatagtatatcggcatagtataatacgacaaggtgaggaactaaatc

SEQ ID NO: 9 - DNA, 1290 bp, Artificial Sequence
  EF1a Genomic
aacccagagatcgctgcgttcccgccccctcacccgcccgctctcgtcatcactgaggtggagaagagcatgcgtgaggctccggtgcccgtcagtgggcagagcgcacatcgcccacagtccccgagaagttggggggaggggtcggcaattgaaccggtgcctagagaaggtggcgcggggtaaactgggaaagtgatgtcgtgtactggctccgcctttttcccgagggtgggggagaaccgtatataagtgcagtagtcgccgtgaacgttctttttcgcaacgggtttgccgccagaacacaggtaagtgccgtgtgtggttcccgcgggcctggcctctttacgggttatggcccttgcgtgccttgaattacttccacgcccctggctgcagtacgtgattcttgatcccgagcttcgggttggaagtgggtgggagagttcgaggccttgcgcttaaggagccccttcgcctcgtgcttgagttgaggcctggcctgggcgctggggccgccgcgtgcgaatctggtggcaccttcgcgcctgtctcgctgctttcgataagtctctagccatttaaaatttttgatgacctgctgcgacgctttttttctggcaagatagtcttgtaaatgcgggccaagatctgcacactggtatttcggtttttggggccgcgggcggcgacggggcccgtgcgtcccagcgcacatgttcggcgaggcggggcctgcgagcgcggccaccgagaatcggacgggggtagtctcaagctggccggcctgctctggtgcctggcctcgcgccgccgtgtatcgccccgccctgggcggcaaggctggcccggtcggcaccagttgcgtgagcggaaagatggccgcttcccggccctgctgcagggagctcaaaatggaggacgcggcgctcgggagagcgggcgggtgagtcacccacacaaaggaaaagggcctttccgtcctcagccgtcgcttcatgtgactccacggagtaccgggcgccgtccaggcacctcgattagttctcgagcttttggagtacgtcgtctttaggttggggggaggggttttatgcgatggagtttccccacactgagtgggtggagactgaagttaggccagcttggcacttgatgtaattctccttggaatttgccctttttgagtttggatcttggttcattctcaagcctcagacagtggttcaaagtttttttcttccatttcaggtgtcgtgaaaactacccctaaaagccaaaatgggaaag

SEQ ID NO: 10 - DNA, 342 bp, Artificial Sequence
  EF1A pPEF
aacccagagatcgctgcgttcccgccccctcacccgcccgctctcgtcatcactgaggtggagaagagcatgcgtgaggctccggtgcccgtcagtgggcagagcgcacatcgcccacagtccccgagaagttggggggaggggtcggcaattgaaccggtgcctagagaaggtggcgcggggtaaactgggaaagtgatgtcgtgtactggctccgcctttttcccgagggtgggggagaaccgtatataagtgcagtagtcgccgtgaacgttctttttcgcaacgggtttgccgccagaacacaggtgtcgtgaaaactacccctaaaagccaaaatgg

SEQ ID NO: 11 - DNA, 1217 bp, Artificial Sequence
  EF1A commercial
agatctcgtgaggctccggtgcccgtcagtgggcagagcgcacatcgcccacagtccccgagaagttggggggaggggtcggcaattgaaccggtgcctagagaaggtggcgcggggtaaactgggaaagtgatgtcgtgtactggctccgcctttttcccgagggtgggggagaaccgtatataagtgcactagtcgccgtgaacgttctttttcgcaacgggtttgccgccagaacacaggtaagtgccgtgtgtggttcccgcgggcctggcctctttacgggttatggcccttgcgtgccttgaattacttccacctggctgcagtacgtgattcttgatcccgagcttcgggttggaagtgggtgggagagttcgtggccttgcgcttaaggagccccttcgcctcgtgcttgagttgtggcctggcctgggcgctggggccgccgcgtgcgaatctggtggcaccttcgcgcctgtctcgctgctttcgataagtctctagccatttaaaatttttgatgacctgctgcgacgctttttttctggcaagatagtcttgtaaatgcgggccaagatcagcacactggtatttcggtttttggggccgcgggcggcgacggggcccgtgcgtcccagcgcacatgttcggcgaggcggggcctgcgagcgcggccaccgagaatcggacgggggtagtctcaagctgcccggcctgctctggtgcctggcctcgcgccgccgtgtatcgccccgccctgggcggcaaggctggcccggtcggcaccagttgcgtgagcggaaagatggccgcttcccggccctgctgcagggagcacaaaatggaggacgcggcgctcgggagagcgggcgggtgagtcacccacacaaaggaaaagggcctttccgtcctcagccgtcgcttcatgtgactccacggagtaccgggcgccgtccaggcacctcgattagttctccagcttttggagtacgtcgtctttaggttggggggaggggttttatgcgatggagtttccccacactgagtgggtggagactgaagttaggccagcttggcacttgatgtaattctccttggaatttgccctttttgagtttggatcttggttcattctcaagcctcagacagtggttcaaagtttttttcttccatttcaggtgtcgtgaaaactacccctaaaagccaaaagatct

SEQ ID NO: 12 - DNA, 1206 bp, Artificial Sequence
  Fragment I with minimal EF1A
gctagccgaggttaactgttgtcctggctgttgcggttccggacaccatcatcaccaccatcaccatcaccattgaggatccagtgtggtggaattctgcagatatccagcacagtggcggccgctcgagtctagagggcccgtttaaacccgctgatcagcctcgactgtgccttctagttgccagccatctgttgtttgcccctcccccgtgccttccttgaccctggaaggtgccactcccactgtcctttcctaataaaatgaggaaattgcatcgcattgtctgagtaggtgtcattctattctggggggtggggtggggcaggacagcaagggggaggattgggaagacaatagcaggcatgctggggatgcggtgggctctatggcttctgaggcggaaagaaccagctggggctctagggggtatccccacgcgccctgtagcggcgcattaagcgcggcgggtgtggtggttacgcaacccagagatcgctgcgttcccgccccctcacccgcccgctctcgtcatcactgaggtggagaagagcatgcgtgaggctccggtgcccgtcagtgggcagagcgcacatcgcccacagtccccgagaagttggggggaggggtcggcaattgaaccggtgcctagagaaggtggcgcggggtaaactgggaaagtgatgtcgtgtactggctccgcctttttcccgagggtgggggagaaccgtatataagtgcagtagtcgccgtgaacgttctttttcgcaacgggtttgccgccagaacacaggtgtcgtgaaaactacccctaaaagcttcaaaatggccaagttgaccagtgccgttccggtgctcaccgcgcgcgacgtcgccggagcggtcgagttctggaccgaccggctcgggttctcccgggacttcgtggaggacgacttcgccggtgtggtccgggacgacgtgaccctgttcatcagcgcggtccaggaccaggtggtgccggacaacaccctggcctgggtgtgggtgcgcggcctggacgagctgtacgccgagtggtcggaggtcgtgtccacgaacttccgggacgcctccgggccggccatgaccgagatcggcgagcagccgtgggggcgggagttcgccctgcgcgacccggccggcaactgcgtgcacttcgtggccgaggagcaggactgacacgtg

SEQ ID NO: 13 - DNA, 1214 bp, Artificial Sequence
  Fragment II with SV40 promoter
gctagccgaggttaactgttgtcctggctgttgcggttccggacaccatcatcaccaccatcaccatcaccattgaggatccagtgtggtggaattctgcagatatccagcacagtggcggccgctcgagtctagagggcccgtttaaacccgctgatcagcctcgactgtgccttctagttgccagccatctgttgtttgcccctcccccgtgccttccttgaccctggaaggtgccactcccactgtcctttcctaataaaatgaggaaattgcatcgcattgtctgagtaggtgtcattctattctggggggtggggtggggcaggacagcaagggggaggattgggaagacaatagcaggcatgctggggatgcggtgggctctatggcttctgaggcggaaagaaccagctggggctctagggggtatccccacgcgccctgtagcggcgcattaagcgcggcgggtgtggtggttacgcctgtggaatgtgtgtcagttagggtgtggaaagtccccaggctccccagcaggcagaagtatgcaaagcatgcatctcaattagtcagcaaccaggtgtggaaagtccccaggctccccagcaggcagaagtatgcaaagcatgcatctcaattagtcagcaaccatagtcccgcccctaactccgcccatcccgcccctaactccgcccagttccgcccattctccgccccatggctgactaattttttttatttatgcagaggccgaggccgcctctgcctctgagctattccagaagtagtgaggaggcttttttggaggcctaggcttttgcaaaaagcttaaaatggccaagttgaccagtgccgttccggtgctcaccgcgcgcgacgtcgccggagcggtcgagttctggaccgaccggctcgggttctcccgggacttcgtggaggacgacttcgccggtgtggtccgggacgacgtgaccctgttcatcagcgcggtccaggaccaggtggtgccggacaacaccctggcctgggtgtgggtgcgcggcctggacgagctgtacgccgagtggtcggaggtcgtgtccacgaacttccgggacgcctccgggccggccatgaccgagatcggcgagcagccgtgggggcgggagttcgccctgcgcgacccggccggcaactgcgtgcacttcgtggccgaggagcaggactgacacgtg

SEQ ID NO: 14 - protein, 315 aa, Artificial Sequence
  N-terminal SUUMOstar secretory tag
HHHHHHHHHHGSLQDSEVNQEAKPEVKPEVKPETHINLKVSDGSSEIFFKIKKTTPLRRLMEAFAKRQGKEMDSLTFLYDGIEIQADQTPEDLDMEDNDIIEAHREQIGGQHYLHIRPAPSDNLPLVDLIEHPDPIFDPKEKDLNETLLRSLLGGHYDPGFMATSPPEDRPGGGGGPAGGAEDLAELDQLLRQRPSGAMPSEIKGLEFSEGLAQGKKQRLSKKLRRKLQMWLWSQTFCPVLYAWNDLGSRFWPRYVKVGSCFSKRSCSVPEGMVCKPSKSVHLTVLRWRCQRRGGQRCGWIPIQYPIISECKCSC

SEQ ID NO: 15 - protein, 352 aa, Artificial Sequence
  Ricin-C3 P2A of PLA2R1
LAEGVAAALTPERLLEWQDKGIFVIQSESLKKCIQAGKSVLTLENCKQANKHMLWKWVSNHGLFNIGGSGCLGLNFSAPEQPLSLYECDSTLVSLRWRCNRKMITGPLQYSVQVAHDNTVVASRKYIHKWISYGSGGGDICEYLHKDLHTIKGNTGSGHHHHHHHHHHRRKRGSGATNFSLLKQAGDVEENPGPQEGWERHGGFCYKIDTVLRSFDQASSGYYCPPALVTITNRFEQAFITSLISSVVKMKDSYFWIALQDQNDTGEYTWKPVGQKPEPVQYTHWNTHQPRYSGGCVAMRGRHPLGRWEVKHCRHFKAMSLCKQPVENQEKAEYEERWPGSGHHHHHHHHHH

SEQ ID NO: 16 - DNA, 346 bp, Artificial Sequence
  pPEF5.2
atataagcagagctcgtttagtgaaccgtcagatctctagaagctgggtaccgaaattaatacgactcactataggggaaccagccaccatgggagtcaaagttctgtttgccctgatctgcatcgctgtggccgaggccaagcccacgctagccgaggttgctttgaggatccagtgtggtggaattctgcagatatccagcacagtggcggccgctcgagtctagagggcccgtttaaacccgctgatcagcctcgactgtgccttctagttgccagccatctgttgtttgcccctcccccgtgccttccttgaccctggaaggtgccactcccactgtccttt

SEQ ID NO: 17 - DNA, 4561 bp, Artificial Sequence
  pPEF5.2
gacggatcgggagatctcccgatcccctatggtcgactctcagtacaatctgctctgatgccgcatagttaagccagtatctgctccctgcttgtgtgttggaggtcgctgagtagtgcgcgagcaaaatttaagctacaacaaggcaaggcttgaccgacaattgcatgaagaatctgcttagggttaggcgttttgcgctgcttcgcgatgtacgggccagatatacgcgttgacattgattattgactagttattaatagtaatcaattacggggtcattagttcatagcccatatatggagttccgcgttacataacttacggtaaatggcccgcctggctgaccgcccaacgacccccgcccattgacgtcaataatgacgtatgttcccatagtaacgccaatagggactttccattgacgtcaatgggtggactatttacggtaaactgcccacttggcagtacatcaagtgtatcatatgccaagtccgccccctattgacgtcaatgacggtaaatggcccgcctggcattatgcccagtacatgaccttacgggactttcctacttggcagtacatctacgtattagtcatcgctattaccatggtgatgcggttttggcagtacaccaatgggcgtggatagcggtttgactcacggggatttccaagtctccaccccattgacgtcaatgggagtttgttttggcaccaaaatcaacgggactttccaaaatgtcgtaataaccccgccccgttgacgcaaatgggcggtaggcgtgtacggtgggaggtctatataagcagagctcgtttagtgaaccgtcagatctctagaagctgggtaccgaaattaatacgactcactataggggaaccagccaccatgggagtcaaagttctgtttgccctgatctgcatcgctgtggccgaggccaagcccacgctagccgaggttgctttgaggatccagtgtggtggaattctgcagatatccagcacagtggcggccgctcgagtctagagggcccgtttaaacccgctgatcagcctcgactgtgccttctagttgccagccatctgttgtttgcccctcccccgtgccttccttgaccctggaaggtgccactcccactgtcctttcctaataaaatgaggaaattgcatcgcattgtctgagtaggtgtcattctattctggggggtggggtggggcaggacagcaagggggaggattgggaagacaatagcaggcatgctggggatgcggtgggctctatggcttctgaggcggaaagaaccagctggggctctagggggtatccccacgcgccctgtagcggcgcattaagcgcggcgggtgtggtggttacgcctgtggaatgtgtgtcagttagggtgtggaaagtccccaggctccccagcaggcagaagtatgcaaagcatgcatctcaattagtcagcaaccaggtgtggaaagtccccaggctccccagcaggcagaagtatgcaaagcatgcatctcaattagtcagcaaccatagtcccgcccctaactccgcccatcccgcccctaactccgcccagttccgcccattctccgccccatggctgactaattttttttatttatgcagaggccgaggccgcctctgcctctgagctattccagaagtagtgaggaggcttttttggaggcctaggcttttgcaaaaagcttaaaatggccaagttgaccagtgccgttccggtgctcaccgcgcgcgacgtcgccggagcggtcgagttctggaccgaccggctcgggttctcccgggacttcgtggaggacgacttcgccggtgtggtccgggacgacgtgaccctgttcatcagcgcggtccaggaccaggtggtgccggacaacaccctggcctgggtgtgggtgcgcggcctggacgagctgtacgccgagtggtcggaggtcgtgtccacgaacttccgggacgcctccgggccggccatgaccgagatcggcgagcagccgtgggggcgggagttcgccctgcgcgacccggccggcaactgcgtgcacttcgtggccgaggagcaggactgacacgtgctacgagatttcgattccaccgccgccttctatgaaaggttgggcttcggaatcgttttccgggacgccggctggatgatcctccagcgcggggatctcatgctggagttcttcgcccaccccaacttgtttattgcagcttataatggttacaaataaagcaatagcatcacaaatttcacaaataaagcatttttttcactgcattctagttgtggtttgtccaaactcatcaatgtatcttatcatgtctgtataccgtcgacctctagctagagcttggcgtaatcatggtcatagctgtttcctgtgtgaaattgttatccgctcacaattccacacaacatacgagccggaagcataaagtgtaaagcctggggtgcctaatgagtgagctaactcacattaattgcgttgcgctcactgcccgctttccagtcgggaaacctgtcgtgccagctgcattaatgaatcggccaacgcgcggggagaggcggtttgcgtattgggcgctcttccgcttcctcgctcactgactcgctgcgctcggtcgttcggctgcggcgagcggtatcagctcactcaaaggcggtaatacggttatccacagaatcaggggataacgcaggaaagaacatgtgagcaaaaggccagcaaaaggccaggaaccgtaaaaaggccgcgttgctggcgtttttccataggctccgcccccctgacgagcatcacaaaaatcgacgctcaagtcagaggtggcgaaacccgacaggactataaagataccaggcgtttccccctggaagctccctcgtgcgctctcctgttccgaccctgccgcttaccggatacctgtccgcctttctcccttcgggaagcgtggcgctttctcaatgctcacgctgtaggtatctcagttcggtgtaggtcgttcgctccaagctgggctgtgtgcacgaaccccccgttcagcccgaccgctgcgccttatccggtaactatcgtcttgagtccaacccggtaagacacgacttatcgccactggcagcagccactggtaacaggattagcagagcgaggtatgtaggcggtgctacagagttcttgaagtggtggcctaactacggctacactagaaggacagtatttggtatctgcgctctgctgaagccagttaccttcggaaaaagagttggtagctcttgatccggcaaacaaaccaccgctggtagcggtggtttttttgtttgcaagcagcagattacgcgcagaaaaaaaggatctcaagaagatcctttgatcttttctacggggtctgacgctcagtggaacgaaaactcacgttaagggattttggtcatgagattatcaaaaaggatcttcacctagatccttttaaattaaaaatgaagttttaaatcaatctaaagtatatatgagtaaacttggtctgacagttaccaatgcttaatcagtgaggcacctatctcagcgatctgtctatttcgttcatccatagttgcctgactccccgtcgtgtagataactacgatacgggagggcttaccatctggccccagtgctgcaatgataccgcgagacccacgctcaccggctccagatttatcagcaataaaccagccagccggaagggccgagcgcagaagtggtcctgcaactttatccgcctccatccagtctattaattgttgccgggaagctagagtaagtagttcgccagttaatagtttgcgcaacgttgttgccattgctacaggcatcgtggtgtcacgctcgtcgtttggtatggcttcattcagctccggttcccaacgatcaaggcgagttacatgatcccccatgttgtgcaaaaaagcggttagctccttcggtcctccgatcgttgtcagaagtaagttggccgcagtgttatcactcatggttatggcagcactgcataattctcttactgtcatgccatccgtaagatgcttttctgtgactggtgagtactcaaccaagtcattctgagaatagtgtatgcggcgaccgagttgctcttgcccggcgtcaatacgggataataccgcgccacatagcagaactttaaaagtgctcatcattggaaaacgttcttcggggcgaaaactctcaaggatcttaccgctgttgagatccagttcgatgtaacccactcgtgcacccaactgatcttcagcatcttttactttcaccagcgtttctgggtgagcaaaaacaggaaggcaaaatgccgcaaaaaagggaataagggcgacacggaaatgttgaatactcatactcttcctttttcaatattattgaagcatttatcagggttattgtctcatgagcggatacatatttgaatgtatttagaaaaataaacaaataggggttccgcgcacatttccccgaaaagtgccacctgacgtc

SEQ ID NO: 18 - DNA, 4746 bp, Artificial Sequence
  pPEF5.2 max
gacggatcgggagatctcccgatcccctatggtcgactctcagtacaatctgctctgatgccgcatagttaagccagtatctgctccctgcttgtgtgttggaggtcgctgagtagtgcgcgagcaaaatttaagctacaacaaggcaaggcttgaccgacaattgcatgaagaatctgcttagggttaggcgttttgcgctgcttcgcgatgtacgggccagatatacgcgttgacattgattattgactagttattaatagtaatcaattacggggtcattagttcatagcccatatatggagttccgcgttacataacttacggtaaatggcccgcctggctgaccgcccaacgacccccgcccattgacgtcaataatgacgtatgttcccatagtaacgccaatagggactttccattgacgtcaatgggtggactatttacggtaaactgcccacttggcagtacatcaagtgtatcatatgccaagtccgccccctattgacgtcaatgacggtaaatggcccgcctggcattatgcccagtacatgaccttacgggactttcctacttggcagtacatctacgtattagtcatcgctattaccatggtgatgcggttttggcagtacaccaatgggcgtggatagcggtttgactcacggggatttccaagtctccaccccattgacgtcaatgggagtttgttttggcaccaaaatcaacgggactttccaaaatgtcgtaataaccccgccccgttgacgcaaatgggcggtaggcgtgtacggtgggaggtctatataagcagagctcgtttagtgaaccgtcagatctctagaagctgggtaccgaaattaatacgactcactatagggagacccaagctggcttgcgtttaaacttaagcttagcgcagaggcttggggcagccgagcggcagccaggccccggcccgggcctcggttccagaagggagaggagcccgccaaggcgcgcaagagagcgggctgcctcgcagtccgagccggagagggagcgcgagccgcgccggccccggacggcctccgaaaccatgggagtcaaagttctgtttgccctgatctgcatcgctgtggccgaggccaagcccacgctagccgaggttgctttgaggatccagtgtggtggaattctgcagatatccagcacagtggcggccgctcgagtctagagggcccgtttaaacccgctgatcagcctcgactgtgccttctagttgccagccatctgttgtttgcccctcccccgtgccttccttgaccctggaaggtgccactcccactgtcctttcctaataaaatgaggaaattgcatcgcattgtctgagtaggtgtcattctattctggggggtggggtggggcaggacagcaagggggaggattgggaagacaatagcaggcatgctggggatgcggtgggctctatggcttctgaggcggaaagaaccagctggggctctagggggtatccccacgcgccctgtagcggcgcattaagcgcggcgggtgtggtggttacgcctgtggaatgtgtgtcagttagggtgtggaaagtccccaggctccccagcaggcagaagtatgcaaagcatgcatctcaattagtcagcaaccaggtgtggaaagtccccaggctccccagcaggcagaagtatgcaaagcatgcatctcaattagtcagcaaccatagtcccgcccctaactccgcccatcccgcccctaactccgcccagttccgcccattctccgccccatggctgactaattttttttatttatgcagaggccgaggccgcctctgcctctgagctattccagaagtagtgaggaggcttttttggaggcctaggcttttgcaaaaagcttaaaatggccaagttgaccagtgccgttccggtgctcaccgcgcgcgacgtcgccggagcggtcgagttctggaccgaccggctcgggttctcccgggacttcgtggaggacgacttcgccggtgtggtccgggacgacgtgaccctgttcatcagcgcggtccaggaccaggtggtgccggacaacaccctggcctgggtgtgggtgcgcggcctggacgagctgtacgccgagtggtcggaggtcgtgtccacgaacttccgggacgcctccgggccggccatgaccgagatcggcgagcagccgtgggggcgggagttcgccctgcgcgacccggccggcaactgcgtgcacttcgtggccgaggagcaggactgacacgtgctacgagatttcgattccaccgccgccttctatgaaaggttgggcttcggaatcgttttccgggacgccggctggatgatcctccagcgcggggatctcatgctggagttcttcgcccaccccaacttgtttattgcagcttataatggttacaaataaagcaatagcatcacaaatttcacaaataaagcatttttttcactgcattctagttgtggtttgtccaaactcatcaatgtatcttatcatgtctgtataccgtcgacctctagctagagcttggcgtaatcatggtcatagctgtttcctgtgtgaaattgttatccgctcacaattccacacaacatacgagccggaagcataaagtgtaaagcctggggtgcctaatgagtgagctaactcacattaattgcgttgcgctcactgcccgctttccagtcgggaaacctgtcgtgccagctgcattaatgaatcggccaacgcgcggggagaggcggtttgcgtattgggcgctcttccgcttcctcgctcactgactcgctgcgctcggtcgttcggctgcggcgagcggtatcagctcactcaaaggcggtaatacggttatccacagaatcaggggataacgcaggaaagaacatgtgagcaaaaggccagcaaaaggccaggaaccgtaaaaaggccgcgttgctggcgtttttccataggctccgcccccctgacgagcatcacaaaaatcgacgctcaagtcagaggtggcgaaacccgacaggactataaagataccaggcgtttccccctggaagctccctcgtgcgctctcctgttccgaccctgccgcttaccggatacctgtccgcctttctcccttcgggaagcgtggcgctttctcaatgctcacgctgtaggtatctcagttcggtgtaggtcgttcgctccaagctgggctgtgtgcacgaaccccccgttcagcccgaccgctgcgccttatccggtaactatcgtcttgagtccaacccggtaagacacgacttatcgccactggcagcagccactggtaacaggattagcagagcgaggtatgtaggcggtgctacagagttcttgaagtggtggcctaactacggctacactagaaggacagtatttggtatctgcgctctgctgaagccagttaccttcggaaaaagagttggtagctcttgatccggcaaacaaaccaccgctggtagcggtggtttttttgtttgcaagcagcagattacgcgcagaaaaaaaggatctcaagaagatcctttgatcttttctacggggtctgacgctcagtggaacgaaaactcacgttaagggattttggtcatgagattatcaaaaaggatcttcacctagatccttttaaattaaaaatgaagttttaaatcaatctaaagtatatatgagtaaacttggtctgacagttaccaatgcttaatcagtgaggcacctatctcagcgatctgtctatttcgttcatccatagttgcctgactccccgtcgtgtagataactacgatacgggagggcttaccatctggccccagtgctgcaatgataccgcgagacccacgctcaccggctccagatttatcagcaataaaccagccagccggaagggccgagcgcagaagtggtcctgcaactttatccgcctccatccagtctattaattgttgccgggaagctagagtaagtagttcgccagttaatagtttgcgcaacgttgttgccattgctacaggcatcgtggtgtcacgctcgtcgtttggtatggcttcattcagctccggttcccaacgatcaaggcgagttacatgatcccccatgttgtgcaaaaaagcggttagctccttcggtcctccgatcgttgtcagaagtaagttggccgcagtgttatcactcatggttatggcagcactgcataattctcttactgtcatgccatccgtaagatgcttttctgtgactggtgagtactcaaccaagtcattctgagaatagtgtatgcggcgaccgagttgctcttgcccggcgtcaatacgggataataccgcgccacatagcagaactttaaaagtgctcatcattggaaaacgttcttcggggcgaaaactctcaaggatcttaccgctgttgagatccagttcgatgtaacccactcgtgcacccaactgatcttcagcatcttttactttcaccagcgtttctgggtgagcaaaaacaggaaggcaaaatgccgcaaaaaagggaataagggcgacacggaaatgttgaatactcatactcttcctttttcaatattattgaagcatttatcagggttattgtctcatgagcggatacatatttgaatgtatttagaaaaataaacaaataggggttccgcgcacatttccccgaaaagtgccacctgacgtc

SEQ ID NO: 19 - DNA, 5223 bp, Artificial Sequence
  pPEF1
gacggatcgggagatctcccgatcccctatggtcgactctcagtacaatctgctctgatgccgcatagttaagccagtatctgctccctgcttgtgtgttggaggtcgctgagtagtgcgcgagcaaaatttaagctacaacaaggcaaggcttgaccgacaattgcatgaagaatctgcttagggttaggcgttttgcgctgcttcgcgatgtacgggccagatatacgcgttgacattgattattgactagttattaatagtaatcaattacggggtcattagttcatagcccatatatggagttccgcgttacataacttacggtaaatggcccgcctggctgaccgcccaacgacccccgcccattgacgtcaataatgacgtatgttcccatagtaacgccaatagggactttccattgacgtcaatgggtggactatttacggtaaactgcccacttggcagtacatcaagtgtatcatatgccaagtccgccccctattgacgtcaatgacggtaaatggcccgcctggcattatgcccagtacatgaccttacgggactttcctacttggcagtacatctacgtattagtcatcgctattaccatggtgatgcggttttggcagtacaccaatgggcgtggatagcggtttgactcacggggatttccaagtctccaccccattgacgtcaatgggagtttgttttggcaccaaaatcaacgggactttccaaaatgtcgtaataaccccgccccgttgacgcaaatgggcggtaggcgtgtacggtgggaggtctatataagcagagctcgtttagtgaaccgtcagatctctagaagctgggtaccgaaattaatacgactcactatagggagacccaagctggcttgcgtttaaacttaagcttagcgcagaggcttggggcagccgagcggcagccaggccccggcccgggcctcggttccagaagggagaggagcccgccaaggcgcgcaagagagcgggctgcctcgcagtccgagccggagagggagcgcgagccgcgccggccccggacggcctccgaaaccatgagggcctggatcttctttctcctttgcctggccgggagggctctggcagccccgctagccgagggatccagtgtggtggaattctgcagatatccagcacagtggcggccgctcgagtctagagggcccgtttaaacccgctgatcagcctcgactgtgccttctagttgccagccatctgttgtttgcccctcccccgtgccttccttgaccctggaaggtgccactcccactgtcctttcctaataaaatgaggaaattgcatcgcattgtctgagtaggtgtcattctattctggggggtggggtggggcaggacagcaagggggaggattgggaagacaatagcaggcatgctggggatgcggtgggctctatggcttctgaggcggaaagaaccagctggggctctagggggtatccccacgcgccctgtagcggcgcattaagcgcggcgggtgtggtggttacgcgcagcgtgaccgctacacttgccagcgccctagcgcccgctcctttcgctttcttcccttcctttctcgccacgttcgccggctttccccgtcaagctctaaatcggggcatccctttagggttccgatttagtgctttacggcacctcgaccccaaaaaacttgattagggtgatggttcacgtagtgggccatcgccctgatagacggtttttcgccctttgacgttggagtccacgttctttaatagtggactcttgttccaaactggaacaacactcaaccctatctcggtctattcttttgatttataagggattttggggatttcggcctattggttaaaaaatgagctgatttaacaaaaatttaacgcgaattaattctgtggaatgtgtgtcagttagggtgtggaaagtccccaggctccccaggcaggcagaagtatgcaaagcatgcatctcaattagtcagcaaccaggtgtggaaagtccccaggctccccagcaggcagaagtatgcaaagcatgcatctcaattagtcagcaaccatagtcccgcccctaactccgcccatcccgcccctaactccgcccagttccgcccattctccgccccatggctgactaattttttttatttatgcagaggccgaggccgcctctgcctctgagctattccagaagtagtgaggaggcttttttggaggcctaggcttttgcaaaaagctcccgggagcttgtatatccattttcggatctgatcagcacgtgttgacaattaatcatcggcatagtatatcggcatagtataatacgacaaggtgaggaactaaaccatggccaagttgaccagtgccgttccggtgctcaccgcgcgcgacgtcgccggagcggtcgagttctggaccgaccggctcgggttctcccgggacttcgtggaggacgacttcgccggtgtggtccgggacgacgtgaccctgttcatcagcgcggtccaggaccaggtggtgccggacaacaccctggcctgggtgtgggtgcgcggcctggacgagctgtacgccgagtggtcggaggtcgtgtccacgaacttccgggacgcctccgggccggccatgaccgagatcggcgagcagccgtgggggcgggagttcgccctgcgcgacccggccggcaactgcgtgcacttcgtggccgaggagcaggactgacacgtgctacgagatttcgattccaccgccgccttctatgaaaggttgggcttcggaatcgttttccgggacgccggctggatgatcctccagcgcggggatctcatgctggagttcttcgcccaccccaacttgtttattgcagcttataatggttacaaataaagcaatagcatcacaaatttcacaaataaagcatttttttcactgcattctagttgtggtttgtccaaactcatcaatgtatcttatcatgtctgtataccgtcgacctctagctagagcttggcgtaatcatggtcatagctgtttcctgtgtgaaattgttatccgctcacaattccacacaacatacgagccggaagcataaagtgtaaagcctggggtgcctaatgagtgagctaactcacattaattgcgttgcgctcactgcccgctttccagtcgggaaacctgtcgtgccagctgcattaatgaatcggccaacgcgcggggagaggcggtttgcgtattgggcgctcttccgcttcctcgctcactgactcgctgcgctcggtcgttcggctgcggcgagcggtatcagctcactcaaaggcggtaatacggttatccacagaatcaggggataacgcaggaaagaacatgtgagcaaaaggccagcaaaaggccaggaaccgtaaaaaggccgcgttgctggcgtttttccataggctccgcccccctgacgagcatcacaaaaatcgacgctcaagtcagaggtggcgaaacccgacaggactataaagataccaggcgtttccccctggaagctccctcgtgcgctctcctgttccgaccctgccgcttaccggatacctgtccgcctttctcccttcgggaagcgtggcgctttctcaatgctcacgctgtaggtatctcagttcggtgtaggtcgttcgctccaagctgggctgtgtgcacgaaccccccgttcagcccgaccgctgcgccttatccggtaactatcgtcttgagtccaacccggtaagacacgacttatcgccactggcagcagccactggtaacaggattagcagagcgaggtatgtaggcggtgctacagagttcttgaagtggtggcctaactacggctacactagaaggacagtatttggtatctgcgctctgctgaagccagttaccttcggaaaaagagttggtagctcttgatccggcaaacaaaccaccgctggtagcggtggtttttttgtttgcaagcagcagattacgcgcagaaaaaaaggatctcaagaagatcctttgatcttttctacggggtctgacgctcagtggaacgaaaactcacgttaagggattttggtcatgagattatcaaaaaggatcttcacctagatccttttaaattaaaaatgaagttttaaatcaatctaaagtatatatgagtaaacttggtctgacagttaccaatgcttaatcagtgaggcacctatctcagcgatctgtctatttcgttcatccatagttgcctgactccccgtcgtgtagataactacgatacgggagggcttaccatctggccccagtgctgcaatgataccgcgagacccacgctcaccggctccagatttatcagcaataaaccagccagccggaagggccgagcgcagaagtggtcctgcaactttatccgcctccatccagtctattaattgttgccgggaagctagagtaagtagttcgccagttaatagtttgcgcaacgttgttgccattgctacaggcatcgtggtgtcacgctcgtcgtttggtatggcttcattcagctccggttcccaacgatcaaggcgagttacatgatcccccatgttgtgcaaaaaagcggttagctccttcggtcctccgatcgttgtcagaagtaagttggccgcagtgttatcactcatggttatggcagcactgcataattctcttactgtcatgccatccgtaagatgcttttctgtgactggtgagtactcaaccaagtcattctgagaatagtgtatgcggcgaccgagttgctcttgcccggcgtcaatacgggataataccgcgccacatagcagaactttaaaagtgctcatcattggaaaacgttcttcggggcgaaaactctcaaggatcttaccgctgttgagatccagttcgatgtaacccactcgtgcacccaactgatcttcagcatcttttactttcaccagcgtttctgggtgagcaaaaacaggaaggcaaaatgccgcaaaaaagggaataagggcgacacggaaatgttgaatactcatactcttcctttttcaatattattgaagcatttatcagggttattgtctcatgagcggatacatatttgaatgtatttagaaaaataaacaaataggggttccgcgcacatttccccgaaaagtgccacctgacgtc

SEQ ID NO: 20 - DNA, 5226 bp, Artificial Sequence
  pPEF2
gacggatcgggagatctcccgatcccctatggtcgactctcagtacaatctgctctgatgccgcatagttaagccagtatctgctccctgcttgtgtgttggaggtcgctgagtagtgcgcgagcaaaatttaagctacaacaaggcaaggcttgaccgacaattgcatgaagaatctgcttagggttaggcgttttgcgctgcttcgcgatgtacgggccagatatacgcgttgacattgattattgactagttattaatagtaatcaattacggggtcattagttcatagcccatatatggagttccgcgttacataacttacggtaaatggcccgcctggctgaccgcccaacgacccccgcccattgacgtcaataatgacgtatgttcccatagtaacgccaatagggactttccattgacgtcaatgggtggactatttacggtaaactgcccacttggcagtacatcaagtgtatcatatgccaagtccgccccctattgacgtcaatgacggtaaatggcccgcctggcattatgcccagtacatgaccttacgggactttcctacttggcagtacatctacgtattagtcatcgctattaccatggtgatgcggttttggcagtacaccaatgggcgtggatagcggtttgactcacggggatttccaagtctccaccccattgacgtcaatgggagtttgttttggcaccaaaatcaacgggactttccaaaatgtcgtaataaccccgccccgttgacgcaaatgggcggtaggcgtgtacggtgggaggtctatataagcagagctcgtttagtgaaccgtcagatctctagaagctgggtaccgaaattaatacgactcactatagggagacccaagctggcttgcgtttaaacttaagcttagcgcagaggcttggggcagccgagcggcagccaggccccggcccgggcctcggttccagaagggagaggagcccgccaaggcgcgcaagagagcgggctgcctcgcagtccgagccggagagggagcgcgagccgcgccggccccggacggcctccgaaaccatgggagtcaaagttctgtttgccctgatctgcatcgctgtggccgaggccaagcccacgctagccgagggatccagtgtggtggaattctgcagatatccagcacagtggcggccgctcgagtctagagggcccgtttaaacccgctgatcagcctcgactgtgccttctagttgccagccatctgttgtttgcccctcccccgtgccttccttgaccctggaaggtgccactcccactgtcctttcctaataaaatgaggaaattgcatcgcattgtctgagtaggtgtcattctattctggggggtggggtggggcaggacagcaagggggaggattgggaagacaatagcaggcatgctggggatgcggtgggctctatggcttctgaggcggaaagaaccagctggggctctagggggtatccccacgcgccctgtagcggcgcattaagcgcggcgggtgtggtggttacgcgcagcgtgaccgctacacttgccagcgccctagcgcccgctcctttcgctttcttcccttcctttctcgccacgttcgccggctttccccgtcaagctctaaatcggggcatccctttagggttccgatttagtgctttacggcacctcgaccccaaaaaacttgattagggtgatggttcacgtagtgggccatcgccctgatagacggtttttcgccctttgacgttggagtccacgttctttaatagtggactcttgttccaaactggaacaacactcaaccctatctcggtctattcttttgatttataagggattttggggatttcggcctattggttaaaaaatgagctgatttaacaaaaatttaacgcgaattaattctgtggaatgtgtgtcagttagggtgtggaaagtccccaggctccccaggcaggcagaagtatgcaaagcatgcatctcaattagtcagcaaccaggtgtggaaagtccccaggctccccagcaggcagaagtatgcaaagcatgcatctcaattagtcagcaaccatagtcccgcccctaactccgcccatcccgcccctaactccgcccagttccgcccattctccgccccatggctgactaattttttttatttatgcagaggccgaggccgcctctgcctctgagctattccagaagtagtgaggaggcttttttggaggcctaggcttttgcaaaaagctcccgggagcttgtatatccattttcggatctgatcagcacgtgttgacaattaatcatcggcatagtatatcggcatagtataatacgacaaggtgaggaactaaaccatggccaagttgaccagtgccgttccggtgctcaccgcgcgcgacgtcgccggagcggtcgagttctggaccgaccggctcgggttctcccgggacttcgtggaggacgacttcgccggtgtggtccgggacgacgtgaccctgttcatcagcgcggtccaggaccaggtggtgccggacaacaccctggcctgggtgtgggtgcgcggcctggacgagctgtacgccgagtggtcggaggtcgtgtccacgaacttccgggacgcctccgggccggccatgaccgagatcggcgagcagccgtgggggcgggagttcgccctgcgcgacccggccggcaactgcgtgcacttcgtggccgaggagcaggactgacacgtgctacgagatttcgattccaccgccgccttctatgaaaggttgggcttcggaatcgttttccgggacgccggctggatgatcctccagcgcggggatctcatgctggagttcttcgcccaccccaacttgtttattgcagcttataatggttacaaataaagcaatagcatcacaaatttcacaaataaagcatttttttcactgcattctagttgtggtttgtccaaactcatcaatgtatcttatcatgtctgtataccgtcgacctctagctagagcttggcgtaatcatggtcatagctgtttcctgtgtgaaattgttatccgctcacaattccacacaacatacgagccggaagcataaagtgtaaagcctggggtgcctaatgagtgagctaactcacattaattgcgttgcgctcactgcccgctttccagtcgggaaacctgtcgtgccagctgcattaatgaatcggccaacgcgcggggagaggcggtttgcgtattgggcgctcttccgcttcctcgctcactgactcgctgcgctcggtcgttcggctgcggcgagcggtatcagctcactcaaaggcggtaatacggttatccacagaatcaggggataacgcaggaaagaacatgtgagcaaaaggccagcaaaaggccaggaaccgtaaaaaggccgcgttgctggcgtttttccataggctccgcccccctgacgagcatcacaaaaatcgacgctcaagtcagaggtggcgaaacccgacaggactataaagataccaggcgtttccccctggaagctccctcgtgcgctctcctgttccgaccctgccgcttaccggatacctgtccgcctttctcccttcgggaagcgtggcgctttctcaatgctcacgctgtaggtatctcagttcggtgtaggtcgttcgctccaagctgggctgtgtgcacgaaccccccgttcagcccgaccgctgcgccttatccggtaactatcgtcttgagtccaacccggtaagacacgacttatcgccactggcagcagccactggtaacaggattagcagagcgaggtatgtaggcggtgctacagagttcttgaagtggtggcctaactacggctacactagaaggacagtatttggtatctgcgctctgctgaagccagttaccttcggaaaaagagttggtagctcttgatccggcaaacaaaccaccgctggtagcggtggtttttttgtttgcaagcagcagattacgcgcagaaaaaaaggatctcaagaagatcctttgatcttttctacggggtctgacgctcagtggaacgaaaactcacgttaagggattttggtcatgagattatcaaaaaggatcttcacctagatccttttaaattaaaaatgaagttttaaatcaatctaaagtatatatgagtaaacttggtctgacagttaccaatgcttaatcagtgaggcacctatctcagcgatctgtctatttcgttcatccatagttgcctgactccccgtcgtgtagataactacgatacgggagggcttaccatctggccccagtgctgcaatgataccgcgagacccacgctcaccggctccagatttatcagcaataaaccagccagccggaagggccgagcgcagaagtggtcctgcaactttatccgcctccatccagtctattaattgttgccgggaagctagagtaagtagttcgccagttaatagtttgcgcaacgttgttgccattgctacaggcatcgtggtgtcacgctcgtcgtttggtatggcttcattcagctccggttcccaacgatcaaggcgagttacatgatcccccatgttgtgcaaaaaagcggttagctccttcggtcctccgatcgttgtcagaagtaagttggccgcagtgttatcactcatggttatggcagcactgcataattctcttactgtcatgccatccgtaagatgcttttctgtgactggtgagtactcaaccaagtcattctgagaatagtgtatgcggcgaccgagttgctcttgcccggcgtcaatacgggataataccgcgccacatagcagaactttaaaagtgctcatcattggaaaacgttcttcggggcgaaaactctcaaggatcttaccgctgttgagatccagttcgatgtaacccactcgtgcacccaactgatcttcagcatcttttactttcaccagcgtttctgggtgagcaaaaacaggaaggcaaaatgccgcaaaaaagggaataagggcgacacggaaatgttgaatactcatactcttcctttttcaatattattgaagcatttatcagggttattgtctcatgagcggatacatatttgaatgtatttagaaaaataaacaaataggggttccgcgcacatttccccgaaaagtgccacctgacgtc

SEQ ID NO: 21 - DNA, 5068 bp, Artificial Sequence
  pPEF3
gacggatcgggagatctcccgatcccctatggtcgactctcagtacaatctgctctgatgccgcatagttaagccagtatctgctccctgcttgtgtgttggaggtcgctgagtagtgcgcgagcaaaatttaagctacaacaaggcaaggcttgaccgacaattgcatgaagaatctgcttagggttaggcgttttgcgctgcttcgcgatgtacgggccagatatacgcgttgacattgattattgactagttattaatagtaatcaattacggggtcattagttcatagcccatatatggagttccgcgttacataacttacggtaaatggcccgcctggctgaccgcccaacgacccccgcccattgacgtcaataatgacgtatgttcccatagtaacgccaatagggactttccattgacgtcaatgggtggactatttacggtaaactgcccacttggcagtacatcaagtgtatcatatgccaagtccgccccctattgacgtcaatgacggtaaatggcccgcctggcattatgcccagtacatgaccttacgggactttcctacttggcagtacatctacgtattagtcatcgctattaccatggtgatgcggttttggcagtacaccaatgggcgtggatagcggtttgactcacggggatttccaagtctccaccccattgacgtcaatgggagtttgttttggcaccaaaatcaacgggactttccaaaatgtcgtaataaccccgccccgttgacgcaaatgggcggtaggcgtgtacggtgggaggtctatataagcagagctcgtttagtgaaccgtcagatctctagaagctgggtaccttaaggcgccagctgatcaagcttctgcctgccgcctgcctgcctgccactgagggttcccagcaccatgagggcctggatcttctttctcctttgcctggccgggagggctctggcagccccgctagccgagggatccagtgtggtggaattctgcagatatccagcacagtggcggccgctcgagtctagagggcccgtttaaacccgctgatcagcctcgactgtgccttctagttgccagccatctgttgtttgcccctcccccgtgccttccttgaccctggaaggtgccactcccactgtcctttcctaataaaatgaggaaattgcatcgcattgtctgagtaggtgtcattctattctggggggtggggtggggcaggacagcaagggggaggattgggaagacaatagcaggcatgctggggatgcggtgggctctatggcttctgaggcggaaagaaccagctggggctctagggggtatccccacgcgccctgtagcggcgcattaagcgcggcgggtgtggtggttacgcgcagcgtgaccgctacacttgccagcgccctagcgcccgctcctttcgctttcttcccttcctttctcgccacgttcgccggctttccccgtcaagctctaaatcggggcatccctttagggttccgatttagtgctttacggcacctcgaccccaaaaaacttgattagggtgatggttcacgtagtgggccatcgccctgatagacggtttttcgccctttgacgttggagtccacgttctttaatagtggactcttgttccaaactggaacaacactcaaccctatctcggtctattcttttgatttataagggattttggggatttcggcctattggttaaaaaatgagctgatttaacaaaaatttaacgcgaattaattctgtggaatgtgtgtcagttagggtgtggaaagtccccaggctccccaggcaggcagaagtatgcaaagcatgcatctcaattagtcagcaaccaggtgtggaaagtccccaggctccccagcaggcagaagtatgcaaagcatgcatctcaattagtcagcaaccatagtcccgcccctaactccgcccatcccgcccctaactccgcccagttccgcccattctccgccccatggctgactaattttttttatttatgcagaggccgaggccgcctctgcctctgagctattccagaagtagtgaggaggcttttttggaggcctaggcttttgcaaaaagctcccgggagcttgtatatccattttcggatctgatcagcacgtgttgacaattaatcatcggcatagtatatcggcatagtataatacgacaaggtgaggaactaaaccatggccaagttgaccagtgccgttccggtgctcaccgcgcgcgacgtcgccggagcggtcgagttctggaccgaccggctcgggttctcccgggacttcgtggaggacgacttcgccggtgtggtccgggacgacgtgaccctgttcatcagcgcggtccaggaccaggtggtgccggacaacaccctggcctgggtgtgggtgcgcggcctggacgagctgtacgccgagtggtcggaggtcgtgtccacgaacttccgggacgcctccgggccggccatgaccgagatcggcgagcagccgtgggggcgggagttcgccctgcgcgacccggccggcaactgcgtgcacttcgtggccgaggagcaggactgacacgtgctacgagatttcgattccaccgccgccttctatgaaaggttgggcttcggaatcgttttccgggacgccggctggatgatcctccagcgcggggatctcatgctggagttcttcgcccaccccaacttgtttattgcagcttataatggttacaaataaagcaatagcatcacaaatttcacaaataaagcatttttttcactgcattctagttgtggtttgtccaaactcatcaatgtatcttatcatgtctgtataccgtcgacctctagctagagcttggcgtaatcatggtcatagctgtttcctgtgtgaaattgttatccgctcacaattccacacaacatacgagccggaagcataaagtgtaaagcctggggtgcctaatgagtgagctaactcacattaattgcgttgcgctcactgcccgctttccagtcgggaaacctgtcgtgccagctgcattaatgaatcggccaacgcgcggggagaggcggtttgcgtattgggcgctcttccgcttcctcgctcactgactcgctgcgctcggtcgttcggctgcggcgagcggtatcagctcactcaaaggcggtaatacggttatccacagaatcaggggataacgcaggaaagaacatgtgagcaaaaggccagcaaaaggccaggaaccgtaaaaaggccgcgttgctggcgtttttccataggctccgcccccctgacgagcatcacaaaaatcgacgctcaagtcagaggtggcgaaacccgacaggactataaagataccaggcgtttccccctggaagctccctcgtgcgctctcctgttccgaccctgccgcttaccggatacctgtccgcctttctcccttcgggaagcgtggcgctttctcaatgctcacgctgtaggtatctcagttcggtgtaggtcgttcgctccaagctgggctgtgtgcacgaaccccccgttcagcccgaccgctgcgccttatccggtaactatcgtcttgagtccaacccggtaagacacgacttatcgccactggcagcagccactggtaacaggattagcagagcgaggtatgtaggcggtgctacagagttcttgaagtggtggcctaactacggctacactagaaggacagtatttggtatctgcgctctgctgaagccagttaccttcggaaaaagagttggtagctcttgatccggcaaacaaaccaccgctggtagcggtggtttttttgtttgcaagcagcagattacgcgcagaaaaaaaggatctcaagaagatcctttgatcttttctacggggtctgacgctcagtggaacgaaaactcacgttaagggattttggtcatgagattatcaaaaaggatcttcacctagatccttttaaattaaaaatgaagttttaaatcaatctaaagtatatatgagtaaacttggtctgacagttaccaatgcttaatcagtgaggcacctatctcagcgatctgtctatttcgttcatccatagttgcctgactccccgtcgtgtagataactacgatacgggagggcttaccatctggccccagtgctgcaatgataccgcgagacccacgctcaccggctccagatttatcagcaataaaccagccagccggaagggccgagcgcagaagtggtcctgcaactttatccgcctccatccagtctattaattgttgccgggaagctagagtaagtagttcgccagttaatagtttgcgcaacgttgttgccattgctacaggcatcgtggtgtcacgctcgtcgtttggtatggcttcattcagctccggttcccaacgatcaaggcgagttacatgatcccccatgttgtgcaaaaaagcggttagctccttcggtcctccgatcgttgtcagaagtaagttggccgcagtgttatcactcatggttatggcagcactgcataattctcttactgtcatgccatccgtaagatgcttttctgtgactggtgagtactcaaccaagtcattctgagaatagtgtatgcggcgaccgagttgctcttgcccggcgtcaatacgggataataccgcgccacatagcagaactttaaaagtgctcatcattggaaaacgttcttcggggcgaaaactctcaaggatcttaccgctgttgagatccagttcgatgtaacccactcgtgcacccaactgatcttcagcatcttttactttcaccagcgtttctgggtgagcaaaaacaggaaggcaaaatgccgcaaaaaagggaataagggcgacacggaaatgttgaatactcatactcttcctttttcaatattattgaagcatttatcagggttattgtctcatgagcggatacatatttgaatgtatttagaaaaataaacaaataggggttccgcgcacatttccccgaaaagtgccacctgacgtc

SEQ ID NO: 22 - DNA, 5041 bp, Artificial Sequence
  pPEF4
gacggatcgggagatctcccgatcccctatggtcgactctcagtacaatctgctctgatgccgcatagttaagccagtatctgctccctgcttgtgtgttggaggtcgctgagtagtgcgcgagcaaaatttaagctacaacaaggcaaggcttgaccgacaattgcatgaagaatctgcttagggttaggcgttttgcgctgcttcgcgatgtacgggccagatatacgcgttgacattgattattgactagttattaatagtaatcaattacggggtcattagttcatagcccatatatggagttccgcgttacataacttacggtaaatggcccgcctggctgaccgcccaacgacccccgcccattgacgtcaataatgacgtatgttcccatagtaacgccaatagggactttccattgacgtcaatgggtggactatttacggtaaactgcccacttggcagtacatcaagtgtatcatatgccaagtccgccccctattgacgtcaatgacggtaaatggcccgcctggcattatgcccagtacatgaccttacgggactttcctacttggcagtacatctacgtattagtcatcgctattaccatggtgatgcggttttggcagtacaccaatgggcgtggatagcggtttgactcacggggatttccaagtctccaccccattgacgtcaatgggagtttgttttggcaccaaaatcaacgggactttccaaaatgtcgtaataaccccgccccgttgacgcaaatgggcggtaggcgtgtacggtgggaggtctatataagcagagctcgtttagtgaaccgtcagatctctagaagctgggtaccgaaattaatacgactcactataggggaaccagccaccatgggagtcaaagttctgtttgccctgatctgcatcgctgtggccgaggccaagcccacgctagccgagggatccagtgtggtggaattctgcagatatccagcacagtggcggccgctcgagtctagagggcccgtttaaacccgctgatcagcctcgactgtgccttctagttgccagccatctgttgtttgcccctcccccgtgccttccttgaccctggaaggtgccactcccactgtcctttcctaataaaatgaggaaattgcatcgcattgtctgagtaggtgtcattctattctggggggtggggtggggcaggacagcaagggggaggattgggaagacaatagcaggcatgctggggatgcggtgggctctatggcttctgaggcggaaagaaccagctggggctctagggggtatccccacgcgccctgtagcggcgcattaagcgcggcgggtgtggtggttacgcgcagcgtgaccgctacacttgccagcgccctagcgcccgctcctttcgctttcttcccttcctttctcgccacgttcgccggctttccccgtcaagctctaaatcggggcatccctttagggttccgatttagtgctttacggcacctcgaccccaaaaaacttgattagggtgatggttcacgtagtgggccatcgccctgatagacggtttttcgccctttgacgttggagtccacgttctttaatagtggactcttgttccaaactggaacaacactcaaccctatctcggtctattcttttgatttataagggattttggggatttcggcctattggttaaaaaatgagctgatttaacaaaaatttaacgcgaattaattctgtggaatgtgtgtcagttagggtgtggaaagtccccaggctccccaggcaggcagaagtatgcaaagcatgcatctcaattagtcagcaaccaggtgtggaaagtccccaggctccccagcaggcagaagtatgcaaagcatgcatctcaattagtcagcaaccatagtcccgcccctaactccgcccatcccgcccctaactccgcccagttccgcccattctccgccccatggctgactaattttttttatttatgcagaggccgaggccgcctctgcctctgagctattccagaagtagtgaggaggcttttttggaggcctaggcttttgcaaaaagctcccgggagcttgtatatccattttcggatctgatcagcacgtgttgacaattaatcatcggcatagtatatcggcatagtataatacgacaaggtgaggaactaaaccatggccaagttgaccagtgccgttccggtgctcaccgcgcgcgacgtcgccggagcggtcgagttctggaccgaccggctcgggttctcccgggacttcgtggaggacgacttcgccggtgtggtccgggacgacgtgaccctgttcatcagcgcggtccaggaccaggtggtgccggacaacaccctggcctgggtgtgggtgcgcggcctggacgagctgtacgccgagtggtcggaggtcgtgtccacgaacttccgggacgcctccgggccggccatgaccgagatcggcgagcagccgtgggggcgggagttcgccctgcgcgacccggccggcaactgcgtgcacttcgtggccgaggagcaggactgacacgtgctacgagatttcgattccaccgccgccttctatgaaaggttgggcttcggaatcgttttccgggacgccggctggatgatcctccagcgcggggatctcatgctggagttcttcgcccaccccaacttgtttattgcagcttataatggttacaaataaagcaatagcatcacaaatttcacaaataaagcatttttttcactgcattctagttgtggtttgtccaaactcatcaatgtatcttatcatgtctgtataccgtcgacctctagctagagcttggcgtaatcatggtcatagctgtttcctgtgtgaaattgttatccgctcacaattccacacaacatacgagccggaagcataaagtgtaaagcctggggtgcctaatgagtgagctaactcacattaattgcgttgcgctcactgcccgctttccagtcgggaaacctgtcgtgccagctgcattaatgaatcggccaacgcgcggggagaggcggtttgcgtattgggcgctcttccgcttcctcgctcactgactcgctgcgctcggtcgttcggctgcggcgagcggtatcagctcactcaaaggcggtaatacggttatccacagaatcaggggataacgcaggaaagaacatgtgagcaaaaggccagcaaaaggccaggaaccgtaaaaaggccgcgttgctggcgtttttccataggctccgcccccctgacgagcatcacaaaaatcgacgctcaagtcagaggtggcgaaacccgacaggactataaagataccaggcgtttccccctggaagctccctcgtgcgctctcctgttccgaccctgccgcttaccggatacctgtccgcctttctcccttcgggaagcgtggcgctttctcaatgctcacgctgtaggtatctcagttcggtgtaggtcgttcgctccaagctgggctgtgtgcacgaaccccccgttcagcccgaccgctgcgccttatccggtaactatcgtcttgagtccaacccggtaagacacgacttatcgccactggcagcagccactggtaacaggattagcagagcgaggtatgtaggcggtgctacagagttcttgaagtggtggcctaactacggctacactagaaggacagtatttggtatctgcgctctgctgaagccagttaccttcggaaaaagagttggtagctcttgatccggcaaacaaaccaccgctggtagcggtggtttttttgtttgcaagcagcagattacgcgcagaaaaaaaggatctcaagaagatcctttgatcttttctacggggtctgacgctcagtggaacgaaaactcacgttaagggattttggtcatgagattatcaaaaaggatcttcacctagatccttttaaattaaaaatgaagttttaaatcaatctaaagtatatatgagtaaacttggtctgacagttaccaatgcttaatcagtgaggcacctatctcagcgatctgtctatttcgttcatccatagttgcctgactccccgtcgtgtagataactacgatacgggagggcttaccatctggccccagtgctgcaatgataccgcgagacccacgctcaccggctccagatttatcagcaataaaccagccagccggaagggccgagcgcagaagtggtcctgcaactttatccgcctccatccagtctattaattgttgccgggaagctagagtaagtagttcgccagttaatagtttgcgcaacgttgttgccattgctacaggcatcgtggtgtcacgctcgtcgtttggtatggcttcattcagctccggttcccaacgatcaaggcgagttacatgatcccccatgttgtgcaaaaaagcggttagctccttcggtcctccgatcgttgtcagaagtaagttggccgcagtgttatcactcatggttatggcagcactgcataattctcttactgtcatgccatccgtaagatgcttttctgtgactggtgagtactcaaccaagtcattctgagaatagtgtatgcggcgaccgagttgctcttgcccggcgtcaatacgggataataccgcgccacatagcagaactttaaaagtgctcatcattggaaaacgttcttcggggcgaaaactctcaaggatcttaccgctgttgagatccagttcgatgtaacccactcgtgcacccaactgatcttcagcatcttttactttcaccagcgtttctgggtgagcaaaaacaggaaggcaaaatgccgcaaaaaagggaataagggcgacacggaaatgttgaatactcatactcttcctttttcaatattattgaagcatttatcagggttattgtctcatgagcggatacatatttgaatgtatttagaaaaataaacaaataggggttccgcgcacatttccccgaaaagtgccacctgacgtc

SEQ ID NO: 23 - DNA, 4553 bp, Artificial Sequence
  pPEF5.1
gacggatcgggagatctcccgatcccctatggtcgactctcagtacaatctgctctgatgccgcatagttaagccagtatctgctccctgcttgtgtgttggaggtcgctgagtagtgcgcgagcaaaatttaagctacaacaaggcaaggcttgaccgacaattgcatgaagaatctgcttagggttaggcgttttgcgctgcttcgcgatgtacgggccagatatacgcgttgacattgattattgactagttattaatagtaatcaattacggggtcattagttcatagcccatatatggagttccgcgttacataacttacggtaaatggcccgcctggctgaccgcccaacgacccccgcccattgacgtcaataatgacgtatgttcccatagtaacgccaatagggactttccattgacgtcaatgggtggactatttacggtaaactgcccacttggcagtacatcaagtgtatcatatgccaagtccgccccctattgacgtcaatgacggtaaatggcccgcctggcattatgcccagtacatgaccttacgggactttcctacttggcagtacatctacgtattagtcatcgctattaccatggtgatgcggttttggcagtacaccaatgggcgtggatagcggtttgactcacggggatttccaagtctccaccccattgacgtcaatgggagtttgttttggcaccaaaatcaacgggactttccaaaatgtcgtaataaccccgccccgttgacgcaaatgggcggtaggcgtgtacggtgggaggtctatataagcagagctcgtttagtgaaccgtcagatctctagaagctgggtaccgaaattaatacgactcactataggggaaccagccaccatgggagtcaaagttctgtttgccctgatctgcatcgctgtggccgaggccaagcccacgctagccgaggttgctttgaggatccagtgtggtggaattctgcagatatccagcacagtggcggccgctcgagtctagagggcccgtttaaacccgctgatcagcctcgactgtgccttctagttgccagccatctgttgtttgcccctcccccgtgccttccttgaccctggaaggtgccactcccactgtcctttcctaataaaatgaggaaattgcatcgcattgtctgagtaggtgtcattctattctggggggtggggtggggcaggacagcaagggggaggattgggaagacaatagcaggcatgctggggatgcggtgggctctatggcttctgaggcggaaagaaccagctggggctctagggggtatccccacgcgccctgtagcggcgcattaagcgcggcgggtgtggtggttacgcaacccagagatcgctgcgttcccgccccctcacccgcccgctctcgtcatcactgaggtggagaagagcatgcgtgaggctccggtgcccgtcagtgggcagagcgcacatcgcccacagtccccgagaagttggggggaggggtcggcaattgaaccggtgcctagagaaggtggcgcggggtaaactgggaaagtgatgtcgtgtactggctccgcctttttcccgagggtgggggagaaccgtatataagtgcagtagtcgccgtgaacgttctttttcgcaacgggtttgccgccagaacacaggtgtcgtgaaaactacccctaaaagcttcaaaatggccaagttgaccagtgccgttccggtgctcaccgcgcgcgacgtcgccggagcggtcgagttctggaccgaccggctcgggttctcccgggacttcgtggaggacgacttcgccggtgtggtccgggacgacgtgaccctgttcatcagcgcggtccaggaccaggtggtgccggacaacaccctggcctgggtgtgggtgcgcggcctggacgagctgtacgccgagtggtcggaggtcgtgtccacgaacttccgggacgcctccgggccggccatgaccgagatcggcgagcagccgtgggggcgggagttcgccctgcgcgacccggccggcaactgcgtgcacttcgtggccgaggagcaggactgacacgtgctacgagatttcgattccaccgccgccttctatgaaaggttgggcttcggaatcgttttccgggacgccggctggatgatcctccagcgcggggatctcatgctggagttcttcgcccaccccaacttgtttattgcagcttataatggttacaaataaagcaatagcatcacaaatttcacaaataaagcatttttttcactgcattctagttgtggtttgtccaaactcatcaatgtatcttatcatgtctgtataccgtcgacctctagctagagcttggcgtaatcatggtcatagctgtttcctgtgtgaaattgttatccgctcacaattccacacaacatacgagccggaagcataaagtgtaaagcctggggtgcctaatgagtgagctaactcacattaattgcgttgcgctcactgcccgctttccagtcgggaaacctgtcgtgccagctgcattaatgaatcggccaacgcgcggggagaggcggtttgcgtattgggcgctcttccgcttcctcgctcactgactcgctgcgctcggtcgttcggctgcggcgagcggtatcagctcactcaaaggcggtaatacggttatccacagaatcaggggataacgcaggaaagaacatgtgagcaaaaggccagcaaaaggccaggaaccgtaaaaaggccgcgttgctggcgtttttccataggctccgcccccctgacgagcatcacaaaaatcgacgctcaagtcagaggtggcgaaacccgacaggactataaagataccaggcgtttccccctggaagctccctcgtgcgctctcctgttccgaccctgccgcttaccggatacctgtccgcctttctcccttcgggaagcgtggcgctttctcaatgctcacgctgtaggtatctcagttcggtgtaggtcgttcgctccaagctgggctgtgtgcacgaaccccccgttcagcccgaccgctgcgccttatccggtaactatcgtcttgagtccaacccggtaagacacgacttatcgccactggcagcagccactggtaacaggattagcagagcgaggtatgtaggcggtgctacagagttcttgaagtggtggcctaactacggctacactagaaggacagtatttggtatctgcgctctgctgaagccagttaccttcggaaaaagagttggtagctcttgatccggcaaacaaaccaccgctggtagcggtggtttttttgtttgcaagcagcagattacgcgcagaaaaaaaggatctcaagaagatcctttgatcttttctacggggtctgacgctcagtggaacgaaaactcacgttaagggattttggtcatgagattatcaaaaaggatcttcacctagatccttttaaattaaaaatgaagttttaaatcaatctaaagtatatatgagtaaacttggtctgacagttaccaatgcttaatcagtgaggcacctatctcagcgatctgtctatttcgttcatccatagttgcctgactccccgtcgtgtagataactacgatacgggagggcttaccatctggccccagtgctgcaatgataccgcgagacccacgctcaccggctccagatttatcagcaataaaccagccagccggaagggccgagcgcagaagtggtcctgcaactttatccgcctccatccagtctattaattgttgccgggaagctagagtaagtagttcgccagttaatagtttgcgcaacgttgttgccattgctacaggcatcgtggtgtcacgctcgtcgtttggtatggcttcattcagctccggttcccaacgatcaaggcgagttacatgatcccccatgttgtgcaaaaaagcggttagctccttcggtcctccgatcgttgtcagaagtaagttggccgcagtgttatcactcatggttatggcagcactgcataattctcttactgtcatgccatccgtaagatgcttttctgtgactggtgagtactcaaccaagtcattctgagaatagtgtatgcggcgaccgagttgctcttgcccggcgtcaatacgggataataccgcgccacatagcagaactttaaaagtgctcatcattggaaaacgttcttcggggcgaaaactctcaaggatcttaccgctgttgagatccagttcgatgtaacccactcgtgcacccaactgatcttcagcatcttttactttcaccagcgtttctgggtgagcaaaaacaggaaggcaaaatgccgcaaaaaagggaataagggcgacacggaaatgttgaatactcatactcttcctttttcaatattattgaagcatttatcagggttattgtctcatgagcggatacatatttgaatgtatttagaaaaataaacaaataggggttccgcgcacatttccccgaaaagtgccacctgacgtc

SEQ ID NO: 24 - DNA, 4738 bp, Artificial Sequence
  pPEF5.1max
gacggatcgggagatctcccgatcccctatggtcgactctcagtacaatctgctctgatgccgcatagttaagccagtatctgctccctgcttgtgtgttggaggtcgctgagtagtgcgcgagcaaaatttaagctacaacaaggcaaggcttgaccgacaattgcatgaagaatctgcttagggttaggcgttttgcgctgcttcgcgatgtacgggccagatatacgcgttgacattgattattgactagttattaatagtaatcaattacggggtcattagttcatagcccatatatggagttccgcgttacataacttacggtaaatggcccgcctggctgaccgcccaacgacccccgcccattgacgtcaataatgacgtatgttcccatagtaacgccaatagggactttccattgacgtcaatgggtggactatttacggtaaactgcccacttggcagtacatcaagtgtatcatatgccaagtccgccccctattgacgtcaatgacggtaaatggcccgcctggcattatgcccagtacatgaccttacgggactttcctacttggcagtacatctacgtattagtcatcgctattaccatggtgatgcggttttggcagtacaccaatgggcgtggatagcggtttgactcacggggatttccaagtctccaccccattgacgtcaatgggagtttgttttggcaccaaaatcaacgggactttccaaaatgtcgtaataaccccgccccgttgacgcaaatgggcggtaggcgtgtacggtgggaggtctatataagcagagctcgtttagtgaaccgtcagatctctagaagctgggtaccgaaattaatacgactcactatagggagacccaagctggcttgcgtttaaacttaagcttagcgcagaggcttggggcagccgagcggcagccaggccccggcccgggcctcggttccagaagggagaggagcccgccaaggcgcgcaagagagcgggctgcctcgcagtccgagccggagagggagcgcgagccgcgccggccccggacggcctccgaaaccatgggagtcaaagttctgtttgccctgatctgcatcgctgtggccgaggccaagcccacgctagccgaggttgctttgaggatccagtgtggtggaattctgcagatatccagcacagtggcggccgctcgagtctagagggcccgtttaaacccgctgatcagcctcgactgtgccttctagttgccagccatctgttgtttgcccctcccccgtgccttccttgaccctggaaggtgccactcccactgtcctttcctaataaaatgaggaaattgcatcgcattgtctgagtaggtgtcattctattctggggggtggggtggggcaggacagcaagggggaggattgggaagacaatagcaggcatgctggggatgcggtgggctctatggcttctgaggcggaaagaaccagctggggctctagggggtatccccacgcgccctgtagcggcgcattaagcgcggcgggtgtggtggttacgcaacccagagatcgctgcgttcccgccccctcacccgcccgctctcgtcatcactgaggtggagaagagcatgcgtgaggctccggtgcccgtcagtgggcagagcgcacatcgcccacagtccccgagaagttggggggaggggtcggcaattgaaccggtgcctagagaaggtggcgcggggtaaactgggaaagtgatgtcgtgtactggctccgcctttttcccgagggtgggggagaaccgtatataagtgcagtagtcgccgtgaacgttctttttcgcaacgggtttgccgccagaacacaggtgtcgtgaaaactacccctaaaagcttcaaaatggccaagttgaccagtgccgttccggtgctcaccgcgcgcgacgtcgccggagcggtcgagttctggaccgaccggctcgggttctcccgggacttcgtggaggacgacttcgccggtgtggtccgggacgacgtgaccctgttcatcagcgcggtccaggaccaggtggtgccggacaacaccctggcctgggtgtgggtgcgcggcctggacgagctgtacgccgagtggtcggaggtcgtgtccacgaacttccgggacgcctccgggccggccatgaccgagatcggcgagcagccgtgggggcgggagttcgccctgcgcgacccggccggcaactgcgtgcacttcgtggccgaggagcaggactgacacgtgctacgagatttcgattccaccgccgccttctatgaaaggttgggcttcggaatcgttttccgggacgccggctggatgatcctccagcgcggggatctcatgctggagttcttcgcccaccccaacttgtttattgcagcttataatggttacaaataaagcaatagcatcacaaatttcacaaataaagcatttttttcactgcattctagttgtggtttgtccaaactcatcaatgtatcttatcatgtctgtataccgtcgacctctagctagagcttggcgtaatcatggtcatagctgtttcctgtgtgaaattgttatccgctcacaattccacacaacatacgagccggaagcataaagtgtaaagcctggggtgcctaatgagtgagctaactcacattaattgcgttgcgctcactgcccgctttccagtcgggaaacctgtcgtgccagctgcattaatgaatcggccaacgcgcggggagaggcggtttgcgtattgggcgctcttccgcttcctcgctcactgactcgctgcgctcggtcgttcggctgcggcgagcggtatcagctcactcaaaggcggtaatacggttatccacagaatcaggggataacgcaggaaagaacatgtgagcaaaaggccagcaaaaggccaggaaccgtaaaaaggccgcgttgctggcgtttttccataggctccgcccccctgacgagcatcacaaaaatcgacgctcaagtcagaggtggcgaaacccgacaggactataaagataccaggcgtttccccctggaagctccctcgtgcgctctcctgttccgaccctgccgcttaccggatacctgtccgcctttctcccttcgggaagcgtggcgctttctcaatgctcacgctgtaggtatctcagttcggtgtaggtcgttcgctccaagctgggctgtgtgcacgaaccccccgttcagcccgaccgctgcgccttatccggtaactatcgtcttgagtccaacccggtaagacacgacttatcgccactggcagcagccactggtaacaggattagcagagcgaggtatgtaggcggtgctacagagttcttgaagtggtggcctaactacggctacactagaaggacagtatttggtatctgcgctctgctgaagccagttaccttcggaaaaagagttggtagctcttgatccggcaaacaaaccaccgctggtagcggtggtttttttgtttgcaagcagcagattacgcgcagaaaaaaaggatctcaagaagatcctttgatcttttctacggggtctgacgctcagtggaacgaaaactcacgttaagggattttggtcatgagattatcaaaaaggatcttcacctagatccttttaaattaaaaatgaagttttaaatcaatctaaagtatatatgagtaaacttggtctgacagttaccaatgcttaatcagtgaggcacctatctcagcgatctgtctatttcgttcatccatagttgcctgactccccgtcgtgtagataactacgatacgggagggcttaccatctggccccagtgctgcaatgataccgcgagacccacgctcaccggctccagatttatcagcaataaaccagccagccggaagggccgagcgcagaagtggtcctgcaactttatccgcctccatccagtctattaattgttgccgggaagctagagtaagtagttcgccagttaatagtttgcgcaacgttgttgccattgctacaggcatcgtggtgtcacgctcgtcgtttggtatggcttcattcagctccggttcccaacgatcaaggcgagttacatgatcccccatgttgtgcaaaaaagcggttagctccttcggtcctccgatcgttgtcagaagtaagttggccgcagtgttatcactcatggttatggcagcactgcataattctcttactgtcatgccatccgtaagatgcttttctgtgactggtgagtactcaaccaagtcattctgagaatagtgtatgcggcgaccgagttgctcttgcccggcgtcaatacgggataataccgcgccacatagcagaactttaaaagtgctcatcattggaaaacgttcttcggggcgaaaactctcaaggatcttaccgctgttgagatccagttcgatgtaacccactcgtgcacccaactgatcttcagcatcttttactttcaccagcgtttctgggtgagcaaaaacaggaaggcaaaatgccgcaaaaaagggaataagggcgacacggaaatgttgaatactcatactcttcctttttcaatattattgaagcatttatcagggttattgtctcatgagcggatacatatttgaatgtatttagaaaaataaacaaataggggttccgcgcacatttccccgaaaagtgccacctgacgtc

SEQ ID NO: 25 - DNA, 9901 bp, Artificial Sequence
  pCEP-Pu/AC7
gccccgccgccggacgaactaaacctgactacggcatctctgccccttcttcgctggtacgaggagcgcttttgttttgtattcggggcagtgcatgtaatcccttcagttggttggtacaacttgccaactgggccctgttccacatgtgacacggggggggaccaaacacaaaggggttctctgactgtagttgacatccttataaatggatgtgcacatttgccaacactgagtggctttcatcctggagcagactttgcatgctgtggactgcaacacaacattgcctttatgtgtaactcttggctgaagctcttacaccaatgctgggggacatgtacctcccaggggcccaggaagactacgggaggctacaccaacgtcaatcagaggggcctgtgtagctaccgataagcggaccctcaagagggcattagcaatagtgtttataaggcccccttgttaaccctaaacgggtagcatatgcttcccgggtagtagtatatactatccagactaaccctaattcaatagcatatgttacccaacgggaagcatatgctatcgaattagggttagtaaaagggtcctaaggaacagcgatatctcccaccccatgagctgtcacggttttatttacatggggtcaggattccacgagggtagtgaaccattttagtcacaagggcagtggctgaagatcaaggagcgggcagtgaactctcctgaatcttcgcctgcttcttcattctccttcgtttagctaatagaataactgctgagttgtgaacagtaaggtgtatgtgaggtgctcgaaaacaaggtttcaggtgacgcccccagaataaaatttggacggggggttcagtggtggcattgtgctatgacaccaatataaccctcacaaaccccttgggcaataaatactagtgtaggaatgaaacattctgaatatctttaacaatagaaatccatggggtggggacaagccgtaaagactggatgtccatctcacacgaatttatggctatgggcaacacataatcctagtgcaatatgatactggggttattaagatgtgtcccaggcagggaccaagacaggtgaaccatgttgttacactctatttgtaacaaggggaaagagagtggacgccgacagcagcggactccactggttgtctctaacacccccgaaaattaaacggggctccacgccaatggggcccataaacaaagacaagtggccactcttttttttgaaattgtggagtgggggcacgcgtcagcccccacacgccgccctgcggttttggactgtaaaataagggtgtaataacttggctgattgtaaccccgctaaccactgcggtcaaaccacttgcccacaaaaccactaatggcaccccggggaatacctgcataagtaggtgggcgggccaagataggggcgcgattgctgcgatctggaggacaaattacacacacttgcgcctgagcgccaagcacagggttgttggtcctcatattcacgaggtcgctgagagcacggtgggctaatgttgccatgggtagcatatactacccaaatatctggatagcatatgctatcctaatctatatctgggtagcataggctatcctaatctatatctgggtagcatatgctatcctaatctatatctgggtagtatatgctatcctaatttatatctgggtagcataggctatcctaatctatatctgggtagcatatgctatcctaatctatatctgggtagtatatgctatcctaatctgtatccgggtagcatatgctatcctaatagagattagggtagtatatgctatcctaatttatatctgggtagcatatactacccaaatatctggatagcatatgctatcctaatctatatctgggtagcatatgctatcctaatctatatctgggtagcataggctatcctaatctatatctgggtagcatatgctatcctaatctatatctgggtagtatatgctatcctaatttatatctgggtagcataggctatcctaatctatatctgggtagcatatgctatcctaatctatatctgggtagtatatgctatcctaatctgtatccgggtagcatatgctatcctcatgcatatacagtcagcatatgatacccagtagtagagtgggagtgctatcctttgcatatgccgccacctcccaagggggcgtgaattttcgctgcttgtccttttcctgcatgctggttgctcccattcttaggtgaatttaaggaggccaggctaaagccgtcgcatgtctgattgctcaccaggtaaatgtcgctaatgttttccaacgcgagaaggtgttgagcgcggagctgagtgacgtgacaacatgggtatgcccaattgccccatgttgggaggacgaaaatggtgacaagacagatggccagaaatacaccaacagcacgcatgatgtctactggggatttattctttagtgcgggggaatacacggcttttaatacgattgagggcgtctcctaacaagttacatcactcctgcccttcctcaccctcatctccatcacctccttcatctccgtcatctccgtcatcaccctccgcggcagccccttccaccataggtggaaaccagggaggcaaatctactccatcgtcaaagctgcacacagtcaccctgatattgcaggtaggagcgggctttgtcataacaaggtccttaatcgcatccttcaaaacctcagcaaatatatgagtttgtaaaaagaccatgaaataacagacaatggactcccttagcgggccaggttgtgggccgggtccaggggccattccaaaggggagacgactcaatggtgtaagacgacattgtggaatagcaagggcagttcctcgccttaggttgtaaagggaggtcttactacctccatatacgaacacaccggcgacccaagttccttcgtcggtagtcctttctacgtgactcctagccaggagagctcttaaaccttctgcaatgttctcaaatttcgggttggaacctccttgaccacgatgctttccaaaccaccctccttttttgcgcctgcctccatcaccctgaccccggggtccagtgcttgggccttctcctgggtcatctgcggggccctgctctatcgctcccgggggcacgtcaggctcaccatctgggccaccttcttggtggtattcaaaataatcggcttcccctacagggtggaaaaatggccttctacctggagggggcctgcgcggtggagacccggatgatgatgactgactactgggactcctgggcctcttttctccacgtccacgacctctccccctggctctttcacgacttccccccctggctctttcacgtcctctaccccggcggcctccactacctcctcgaccccggcctccactacctcctcgaccccggcctccactgcctcctcgaccccggcctccacctcctgctcctgcccctcctgctcctgcccctcctcctgctcctgcccctcctgcccctcctgctcctgcccctcctgcccctcctgctcctgcccctcctgcccctcctgctcctgcccctcctgcccctcctcctgctcctgcccctcctgcccctcctcctgctcctgcccctcctgcccctcctgctcctgcccctcctgcccctcctgctcctgcccctcctgcccctcctgctcctgcccctcctgctcctgcccctcctgctcctgcccctcctgctcctgcccctcctgcccctcctgcccctcctcctgctcctgcccctcctgctcctgcccctcctgcccctcctgcccctcctgctcctgcccctcctcctgctcctgcccctcctgcccctcctgcccctcctcctgctcctgcccctcctgcccctcctcctgctcctgcccctcctcctgctcctgcccctcctgcccctcctgcccctcctcctgctcctgcccctcctgcccctcctcctgctcctgcccctcctcctgctcctgcccctcctgcccctcctgcccctcctcctgctcctgcccctcctcctgctcctgcccctcctgcccctcctgcccctcctgcccctcctcctgctcctgcccctcctcctgctcctgcccctcctgctcctgcccctcccgctcctgctcctgctcctgttccaccgtgggtccctttgcagccaatgcaacttggacgtttttggggtctccggacaccatctctatgtcttggccctgatcctgagccgcccggggctcctggtcttccgcctcctcgtcctcgtcctcttccccgtcctcgtccatggttatcaccccctcttctttgaggtccactgccgccggagccttctggtccagatgtgtctcccttctctcctaggccatttccaggtcctgtacctggcccctcgtcagacatgattcacactaaaagagatcaatagacatctttattagacgacgctcagtgaatacagggagtgcagactcctgccccctccaacagcccccccaccctcatccccttcatggtcgctgtcagacagatccaggtctgaaaattccccatcctccgaaccatcctcgtcctcatcaccaattactcgcagcccggaaaactcccgctgaacatcctcaagatttgcgtcctgagcctcaagccaggcctcaaattcctcgtccccctttttgctggacggtagggatggggattctcgggacccctcctcttcctcttcaaggtcaccagacagagatgctactggggcaacggaagaaaagctgggtgcggcctgtgaggatcagcttatcgatgataagctgtcaaacatgagaattcttgaagacgaaagggcctcgtgatacgcctatttttataggttaatgtcatgataataatggtttcttagacgtcaggtggcacttttcggggaaatgtgcgcggaacccctatttgtttatttttctaaatacattcaaatatgtatccgctcatgagacaataaccctgataaatgcttcaataatattgaaaaaggaagagtatgagtattcaacatttccgtgtcgcccttattcccttttttgcggcattttgccttcctgtttttgctcacccagaaacgctggtgaaagtaaaagatgctgaagatcagttgggtgcacgagtgggttacatcgaactggatctcaacagcggtaagatccttgagagttttcgccccgaagaacgttttccaatgatgagcacttttaaagttctgctatgtggcgcggtattatcccgtgttgacgccgggcaagagcaactcggtcgccgcatacactattctcagaatgacttggttgagtactcaccagtcacagaaaagcatcttacggatggcatgacagtaagagaattatgcagtgctgccataaccatgagtgataacactgcggccaacttacttctgacaacgatcggaggaccgaaggagctaaccgcttttttgcacaacatgggggatcatgtaactcgccttgatcgttgggaaccggagctgaatgaagccataccaaacgacgagcgtgacaccacgatgcctgcagcaatggcaacaacgttgcgcaaactattaactggcgaactacttactctagcttcccggcaacaattaatagactggatggaggcggataaagttgcaggaccacttctgcgctcggcccttccggctggctggtttattgctgataaatctggagccggtgagcgtgggtctcgcggtatcattgcagcactggggccagatggtaagccctcccgtatcgtagttatctacacgacggggagtcaggcaactatggatgaacgaaatagacagatcgctgagataggtgcctcactgattaagcattggtaactgtcagaccaagtttactcatatatactttagattgatttaaaacttcatttttaatttaaaaggatctaggtgaagatcctttttgataatctcatgaccaaaatcccttaacgtgagttttcgttccactgagcgtcagaccccgtagaaaagatcaaaggatcttcttgagatcctttttttctgcgcgtaatctgctgcttgcaaacaaaaaaaccaccgctaccagcggtggtttgtttgccggatcaagagctaccaactctttttccgaaggtaactggcttcagcagagcgcagataccaaatactgtccttctagtgtagccgtagttaggccaccacttcaagaactctgtagcaccgcctacatacctcgctctgctaatcctgttaccagtggctgctgccagtggcgataagtcgtgtcttaccgggttggactcaagacgatagttaccggataaggcgcagcggtcgggctgaacggggggttcgtgcacacagcccagcttggagcgaacgacctacaccgaactgagatacctacagcgtgagctatgagaaagcgccacgcttcccgaagggagaaaggcggacaggtatccggtaagcggcagggtcggaacaggagagcgcacgagggagcttccagggggaaacgcctggtatctttatagtcctgtcgggtttcgccacctctgacttgagcgtcgatttttgtgatgctcgtcaggggggcggagcctatggaaaaacgccagcaacgcggcctttttacggttcctggccttttgctgcgccgcgtgcggctgctggagatggcggacgcgatggatatgttctgccaagggttggtttgcgcattcacagttctccgcaagaattgattggctccaattcttggagtggtgaatccgttagcgaggccatccagcctcgcgtcgaactagatgatccgctgtggaatgtgtgtcagttagggtgtggaaagtccccaggctccccagcaggcagaagtatgcaaagcatgcatctcaattagtcagcaaccaggtgtggaaagtccccaggctccccagcaggcagaagtatgcaaagcatgcatctcaattagtcagcaaccatagtcccgcccctaactccgcccatcccgcccctaactccgcccagttccgcccattctccgccccatggctgactaattttttttatttatgcagaggccgaggccgcctcggcctctgagctattccagaagtagtgaggaggcttttttggagggtgaccgccacgaccggtgccgccaccatcccctgacccacgcccctgacccctcacaaggagacgaccttccatgaccgagtacaagcccacggtgcgcctcgccacccgcgacgacgtcccccgggccgtacgcaccctcgccgccgcgttcgccgactaccccgccacgcgccacaccgtcgaccccgaccgccacatcgaacgcgtcaccgagctgcaagaactcttcctcacgcgcgtcgggctcgacatcggcaaggtgtgggtcgcggacgacggcgccgcggtggcggtctggaccacgccggagagcgtcgaagcgggggcggtgttcgccgagatcggcccgcgcatggccgagttgagcggttcccggctggccgcgcagcaacagatggaaggcctcctggcgccgcaccggcccaaggagcccgcgtggttcctggccaccgtcggcgtctcgcccgaccaccagggcaagggtctgggcagcgccgtcgtgctccccggagtggaggcggccgagcgcgccggggtgcccgccttcctggagacctccgcgccccgcaacctccccttctacgagcggctcggcttcaccgtcaccgccgacgtcgagtgcccgaaggaccgcgcgacctggtgcatgacccgcaagcccggtgcctgacgcccgccccacgacccgcagcgcccgaccgaaaggagcgcacgacccggtccgacggcggcccacgggtcccaggggggtcgacctcgaaacttgtttattgcagcttataatggttacaaataaagcaatagcatcacaaatttcacaaataaagcatttttttcactgcattctagttgtggtttgtccaaactcatcaatgtatcttatcatgtctggatcgatccgaaccccttcctcgaccaattctcatgtttgacagcttatcatcgcagatccgggcaacgttgttgcattgctgcaggcgcagaactggtaggtatggaagatctatacattgaatcaatattggcaattagccatattagtcattggttatatagcataaatcaatattggctattggccattgcatacgttgtatctatatcataatatgtacatttatattggctcatgtccaatatgaccgccatgttgacattgattattgactagttattaatagtaatcaattacggggtcattagttcatagcccatatatggagttccgcgttacataacttacggtaaatggcccgcctggctgaccgcccaacgacccccgcccattgacgtcaataatgacgtatgttcccatagtaacgccaatagggactttccattgacgtcaatgggtggagtatttacggtaaactgcccacttggcagtacatcaagtgtatcatatgccaagtccgccccctattgacgtcaatgacggtaaatggcccgcctggcattatgcccagtacatgaccttacgggactttcctacttggcagtacatctacgtattagtcatcgctattaccatggtgatgcggttttggcagtacaccaatgggcgtggatagcggtttgactcacggggatttccaagtctccaccccattgacgtcaatgggagtttgttttggcaccaaaatcaacgggactttccaaaatgtcgtaataaccccgccccgttgacgcaaatgggcggtaggcgtgtacggtgggaggtctatataagcagagctcgtttagtgaaccgtcagatctctagaagctgggtaccttaaggcgccagctgatcaagcttctgcctgccgcctgcctgcctgccactgagggttcccagcaccatgagggcctggatcttctttctcctttgcctggccgggagggctctggcagccccgctagctctcactgaaacagatatatgcaagttgccgaaagacgaaggaacttgcagggatttcatattaaaatggtactatgatccaaacaccaaaagctgtgcaagattctggtatggaggttgtggtggaaacgaaaacaaatttggatcacagaaagaatgtgaaaaggtttgcgctcctgtgctcgccaaacccggagtcatcagtgtgatgggaacctaagcgtgggtggccaacatcatatacctcttgaagaagaaggagtcagccatcgccaacttgtctcgaggtccgcggccgctcgaggccggcaaggccggatccagacatgataagatacattgatgagtttggacaaaccacaactagaatgcagtgaaaaaaatgctttatttgtgaaatttgtgatgctattgctttatttgtaaccattataagctgcaataaacaagttaacaacaacaattgcattcattttatgtttcaggttcagggggaggtggggaggttttttaaagcaagtaaaacctctacaaatgtggtatggctgattatgatccggctgcctcgcgcgtttcggtgatgacggtgaaaacctctgacacatgcagctcccggagacggtcacagcttgtctgtaagcggatgccgggagcagacaagcccgtcagggcgcgtcagcgggtgttggcgggtgtcggggcgcagccatgaccggtcgactctaga

SEQ ID NO: 26 - DNA, 163 bp, Artificial Sequence
  QBI SP163 translational enhancer
agcgcagaggcttggggcagccgagcggcagccaggccccggcccgggcctcggttccagaagggagaggagcccgccaaggcgcgcaagagagcgggctgcctcgcagtccgagccggagagggagcgcgagccgcgccggccccggacggcctccgaaacc

SEQ ID NO: 27 - DNA, 73 bp, Artificial Sequence
  Polylinker/MCS
acgctagccgaggttaactgttgtcctggctgttgcggttccggacaccatcatcaccaccatcaccatcacc

SEQ ID NO: 28 - DNA, 77 bp, Artificial Sequence
  Polylinker/MCS
attgaggatccagtgtggtggaattctgcagatatccagcacagtggcggccgctcgagtctagagggcccgtttaa

SEQ ID NO: 29 - DNA, 73 bp, Artificial Sequence
  Polylinker/MCS
acgctagccgaggttgctttgaggatccagtgtggtggaattctgcagatatccagcacagtggcggccgctc

SEQ ID NO: 30 - DNA, 21 bp, Artificial Sequence
  31
gagtctagagggcccgtttaa

SEQ ID NO: 31 - DNA, 344 bp, Artificial Sequence
  SV40 promoter
ctgtggaatgtgtgtcagttagggtgtggaaagtccccaggctccccagcaggcagaagtatgcaaagcatgcatctcaattagtcagcaaccaggtgtggaaagtccccaggctccccagcaggcagaagtatgcaaagcatgcatctcaattagtcagcaaccatagtcccgcccctaactccgcccatcccgcccctaactccgcccagttccgcccattctccgccccatggctgactaattttttttatttatgcagaggccgaggccgcctctgcctctgagctattccagaagtagtgaggaggcttttttggaggcctaggcttttgcaaaaagct

SEQ ID NO: 32 - DNA, 577 bp, Artificial Sequence
  CMV immediate early promoter
acattgattattgactagttattaatagtaatcaattacggggtcattagttcatagcccatatatggagttccgcgttacataacttacggtaaatggcccgcctggctgaccgcccaacgacccccgcccattgacgtcaataatgacgtatgttcccatagtaacgccaatagggactttccattgacgtcaatgggtggactatttacggtaaactgcccacttggcagtacatcaagtgtatcatatgccaagtccgccccctattgacgtcaatgacggtaaatggcccgcctggcattatgcccagtacatgaccttacgggactttcctacttggcagtacatctacgtattagtcatcgctattaccatggtgatgcggttttggcagtacaccaatgggcgtggatagcggtttgactcacggggatttccaagtctccaccccattgacgtcaatgggagtttgttttggcaccaaaatcaacgggactttccaaaatgtcgtaataaccccgccccgttgacgcaaatgggcggtaggcgtgtacggtgggaggtctatataagc

SEQ ID NO: 33 - DNA, 342 bp, Artificial Sequence; identical to SEQ ID NO: 10
  EF1 alpha promoter minimal

SEQ ID NO: 34 - DNA, 1285 bp, Artificial Sequence
  EF1 alpha promoter genomic
aacccagagatcgctgcgttcccgccccctcacccgcccgctctcgtcatcactgaggtggagaagagcatgcgtgaggctccggtgcccgtcagtgggcagagcgcacatcgcccacagtccccgagaagttggggggaggggtcggcaattgaaccggtgcctagagaaggtggcgcggggtaaactgggaaagtgatgtcgtgtactggctccgcctttttcccgagggtgggggagaaccgtatataagtgcagtagtcgccgtgaacgttctttttcgcaacgggtttgccgccagaacacaggtaagtgccgtgtgtggttcccgcgggcctggcctctttacgggttatggcccttgcgtgccttgaattacttccacgcccctggctgcagtacgtgattcttgatcccgagcttcgggttggaagtgggtgggagagttcgaggccttgcgcttaaggagccccttcgcctcgtgcttgagttgaggcctggcctgggcgctggggccgccgcgtgcgaatctggtggcaccttcgcgcctgtctcgctgctttcgataagtctctagccatttaaaatttttgatgacctgctgcgacgctttttttctggcaagatagtcttgtaaatgcgggccaagatctgcacactggtatttcggtttttggggccgcgggcggcgacggggcccgtgcgtcccagcgcacatgttcggcgaggcggggcctgcgagcgcggccaccgagaatcggacgggggtagtctcaagctggccggcctgctctggtgcctggcctcgcgccgccgtgtatcgccccgccctgggcggcaaggctggcccggtcggcaccagttgcgtgagcggaaagatggccgcttcccggccctgctgcagggagctcaaaatggaggacgcggcgctcgggagagcgggcgggtgagtcacccacacaaaggaaaagggcctttccgtcctcagccgtcgcttcatgtgactccacggagtaccgggcgccgtccaggcacctcgattagttctcgagcttttggagtacgtcgtctttaggttggggggaggggttttatgcgatggagtttccccacactgagtgggtggagactgaagttaggccagcttggcacttgatgtaattctccttggaatttgccctttttgagtttggatcttggttcattctcaagcctcagacagtggttcaaagtttttttcttccatttcaggtgtcgtgaaaactacccctaaaagccaaaatgg

SEQ ID NO: 35 - DNA, 1217 bp, Artificial Sequence; identical to SEQ ID NO: 11
  EF1 alpha promoter commercial

SEQ ID NO: 36 - DNA, 122 bp, Artificial Sequence
  Deletion fragment of MCS primer
cgctgtggccgaggccaagcccacgctagccgaggttaactgttgtcctggctgttgcggttccggacaccatcatcaccaccatcaccatcaccattgaggatccagtgtggtggaattct

SEQ ID NO: 37 - DNA, 21 bp, Artificial Sequence
  pPEF5.2 reverse primer
caacagccaggacaacagtta

SEQ ID NO: 38 - DNA, 30 bp, Artificial Sequence
  pPEF5.2 Forward primer introducing AfeI
ggtgagcgctttgaggatccagtgtggtgg

SEQ ID NO: 39 - DNA, 901 bp, Artificial Sequence
  Synthetic PuroR DNA
caaagcatgcatctcaattagtcagcaaccaggtgtggaaagtccccaggctccccagcaggcagaagtatgcaaagcatgcatctcaattagtcagcaaccatagtcccgcccctaactccgcccatcccgcccctaactccgcccagttccgcccattctccgccccatggctgactaattttttttatttatgcagaggccgaggccgcctctgcctctgagctattccagaagtagtgaggaggcttttttggaggcctaggcttttgcaaaaagcttgaggaactaaaccatgaccgagtacaagcccacggtgcgcctcgccacccgcgacgacgtccccagggccgtacgcaccctcgccgccgcgttcgccgactaccccgccacgcgccacaccgtcgatccggaccgccacatcgagcgggtcaccgagctgcaagaactcttcctcacgcgcgtcgggctcgacatcggcaaggtgtgggtcgcggacgacggcgccgcggtggcggtctggaccacgccggagagcgtcgaagcgggggcggtgttcgccgagatcggcccgcgcatggccgagttgagcggttcccggctggccgcgcagcaacagatggaaggcctcctggcgccgcaccggcccaaggagcccgcgtggttcctggccaccgtcggcgtctcgcccgaccaccagggcaagggtctgggcagcgccgtcgtgctccccggagtggaggcggccgagcgcgccggggtgcccgccttcctggagacatccgcgccccgcaacctccccttctacgagcggctcggcttcaccgtcaccgccgacgtcgaggtgcccgaaggaccgcgcacctggtgcatgacccgcaagcccggtgcctgacacgtg

SEQ ID NO: 40 - DNA, 4802 bp, Artificial Sequence
  pPEF5PuroR
gacggatcgggagatctcccgatcccctatggtcgactctcagtacaatctgctctgatgccgcatagttaagccagtatctgctccctgcttgtgtgttggaggtcgctgagtagtgcgcgagcaaaatttaagctacaacaaggcaaggcttgaccgacaattgcatgaagaatctgcttagggttaggcgttttgcgctgcttcgcgatgtacgggccagatatacgcgttgacattgattattgactagttattaatagtaatcaattacggggtcattagttcatagcccatatatggagttccgcgttacataacttacggtaaatggcccgcctggctgaccgcccaacgacccccgcccattgacgtcaataatgacgtatgttcccatagtaacgccaatagggactttccattgacgtcaatgggtggactatttacggtaaactgcccacttggcagtacatcaagtgtatcatatgccaagtccgccccctattgacgtcaatgacggtaaatggcccgcctggcattatgcccagtacatgaccttacgggactttcctacttggcagtacatctacgtattagtcatcgctattaccatggtgatgcggttttggcagtacaccaatgggcgtggatagcggtttgactcacggggatttccaagtctccaccccattgacgtcaatgggagtttgttttggcaccaaaatcaacgggactttccaaaatgtcgtaataaccccgccccgttgacgcaaatgggcggtaggcgtgtacggtgggaggtctatataagcagagctcgtttagtgaaccgtcagatctctagaagctgggtaccgaaattaatacgactcactataggggaaccagccaccatgggagtcaaagttctgtttgccctgatctgcatcgctgtggccgaggccaagcccacgctagccgaggttgctttgaggatccagtgtggtggaattctgcagatatccagcacagtggcggccgctcgagtctagagggcccgtttaaacccgctgatcagcctcgactgtgccttctagttgccagccatctgttgtttgcccctcccccgtgccttccttgaccctggaaggtgccactcccactgtcctttcctaataaaatgaggaaattgcatcgcattgtctgagtaggtgtcattctattctggggggtggggtggggcaggacagcaagggggaggattgggaagacaatagcaggcatgctggggatgcggtgggctctatggcttctgaggcggaaagaaccagctggggctctagggggtatccccacgcgccctgtagcggcgcattaagcgcggcgggtgtggtggttacgcctgtggaatgtgtgtcagttagggtgtggaaagtccccaggctccccagcaggcagaagtatgcaaagcatgcatctcaattagtcagcaaccaggtgtggaaagtccccaggctccccagcaggcagaagtatgcaaagcatgcatctcaattagtcagcaaccatagtcccgcccctaactccgcccatcccgcccctaactccgcccagttccgcccattctccgccccatggctgactaattttttttatttatgcagaggccgaggccgcctctgcctctgagctattccagaagtagtgaggaggcttttttggaggcctaggcttttgcaaaaagcttgaggaactaaaccatgaccgagtacaagcccacggtgcgcctcgccacccgcgacgacgtccccagggccgtacgcaccctcgccgccgcgttcgccgactaccccgccacgcgccacaccgtcgatccggaccgccacatcgagcgggtcaccgagctgcaagaactcttcctcacgcgcgtcgggctcgacatcggcaaggtgtgggtcgcggacgacggcgccgcggtggcggtctggaccacgccggagagcgtcgaagcgggggcggtgttcgccgagatcggcccgcgcatggccgagttgagcggttcccggctggccgcgcagcaacagatggaaggcctcctggcgccgcaccggcccaaggagcccgcgtggttcctggccaccgtcggcgtctcgcccgaccaccagggcaagggtctgggcagcgccgtcgtgctccccggagtggaggcggccgagcgcgccggggtgcccgccttcctggagacatccgcgccccgcaacctccccttctacgagcggctcggcttcaccgtcaccgccgacgtcgaggtgcccgaaggaccgcgcacctggtgcatgacccgcaagcccggtgcctgacacgtgaaagtgctacgagatttcgattccaccgccgccttctatgaaaggttgggcttcggaatcgttttccgggacgccggctggatgatcctccagcgcggggatctcatgctggagttcttcgcccaccccaacttgtttattgcagcttataatggttacaaataaagcaatagcatcacaaatttcacaaataaagcatttttttcactgcattctagttgtggtttgtccaaactcatcaatgtatcttatcatgtctgtataccgtcgacctctagctagagcttggcgtaatcatggtcatagctgtttcctgtgtgaaattgttatccgctcacaattccacacaacatacgagccggaagcataaagtgtaaagcctggggtgcctaatgagtgagctaactcacattaattgcgttgcgctcactgcccgctttccagtcgggaaacctgtcgtgccagctgcattaatgaatcggccaacgcgcggggagaggcggtttgcgtattgggcgctcttccgcttcctcgctcactgactcgctgcgctcggtcgttcggctgcggcgagcggtatcagctcactcaaaggcggtaatacggttatccacagaatcaggggataacgcaggaaagaacatgtgagcaaaaggccagcaaaaggccaggaaccgtaaaaaggccgcgttgctggcgtttttccataggctccgcccccctgacgagcatcacaaaaatcgacgctcaagtcagaggtggcgaaacccgacaggactataaagataccaggcgtttccccctggaagctccctcgtgcgctctcctgttccgaccctgccgcttaccggatacctgtccgcctttctcccttcgggaagcgtggcgctttctcaatgctcacgctgtaggtatctcagttcggtgtaggtcgttcgctccaagctgggctgtgtgcacgaaccccccgttcagcccgaccgctgcgccttatccggtaactatcgtcttgagtccaacccggtaagacacgacttatcgccactggcagcagccactggtaacaggattagcagagcgaggtatgtaggcggtgctacagagttcttgaagtggtggcctaactacggctacactagaaggacagtatttggtatctgcgctctgctgaagccagttaccttcggaaaaagagttggtagctcttgatccggcaaacaaaccaccgctggtagcggtggtttttttgtttgcaagcagcagattacgcgcagaaaaaaaggatctcaagaagatcctttgatcttttctacggggtctgacgctcagtggaacgaaaactcacgttaagggattttggtcatgagattatcaaaaaggatcttcacctagatccttttaaattaaaaatgaagttttaaatcaatctaaagtatatatgagtaaacttggtctgacagttaccaatgcttaatcagtgaggcacctatctcagcgatctgtctatttcgttcatccatagttgcctgactccccgtcgtgtagataactacgatacgggagggcttaccatctggccccagtgctgcaatgataccgcgagacccacgctcaccggctccagatttatcagcaataaaccagccagccggaagggccgagcgcagaagtggtcctgcaactttatccgcctccatccagtctattaattgttgccgggaagctagagtaagtagttcgccagttaatagtttgcgcaacgttgttgccattgctacaggcatcgtggtgtcacgctcgtcgtttggtatggcttcattcagctccggttcccaacgatcaaggcgagttacatgatcccccatgttgtgcaaaaaagcggttagctccttcggtcctccgatcgttgtcagaagtaagttggccgcagtgttatcactcatggttatggcagcactgcataattctcttactgtcatgccatccgtaagatgcttttctgtgactggtgagtactcaaccaagtcattctgagaatagtgtatgcggcgaccgagttgctcttgcccggcgtcaatacgggataataccgcgccacatagcagaactttaaaagtgctcatcattggaaaacgttcttcggggcgaaaactctcaaggatcttaccgctgttgagatccagttcgatgtaacccactcgtgcacccaactgatcttcagcatcttttactttcaccagcgtttctgggtgagcaaaaacaggaaggcaaaatgccgcaaaaaagggaataagggcgacacggaaatgttgaatactcatactcttcctttttcaatattattgaagcatttatcagggttattgtctcatgagcggatacatatttgaatgtatttagaaaaataaacaaataggggttccgcgcacatttccccgaaaagtgccacctgacgtc

SEQ ID NO: 41 - DNA, 290 bp, Artificial Sequence
  Minimal EF1A1
cctcacccgcccgctctcgtcatcactgaggtggagaagagcatgcgtgaggctccggtgcccgtcagtgggcagagcgcacatcgcccacagtccccgagaagttggggggaggggtcggcaattgaaccggtgcctagagaaggtggcgcggggtaaactgggaaagtgatgtcgtgtactggctccgcctttttcccgagggtgggggagaaccgtatataagtgcagtagtcgccgtgaacgttctttttcgcaacgggtttgccgccagaacacaggtgtcgtga

SEQ ID NO: 42 - DNA, 156 bp, Artificial Sequence
  Minimal EF1A2
gcctagagaaggtggcgcggggtaaactgggaaagtgatgtcgtgtactggctccgcctttttcccgagggtgggggagaaccgtatataagtgcagtagtcgccgtgaacgttctttttcgcaacgggtttgccgccagaacacaggtgtcgtga

SEQ ID NO: 43 - DNA, 157 bp, Artificial Sequence
  Minimal EF1A3
aacccagagatcgctgcgttcccgccccctcacccgcccgctctcgtcatcactgagcctttttcccgagggtgggggagaaccgtatataagtgcagtagtcgccgtgaacgttctttttcgcaacgggtttgccgccagaacacaggtgtcgtga

SEQ ID NO: 44 - DNA, 26 bp, Artificial Sequence
  Forward primer EF_Forward1
tttaggcctcacccgcccgctctcgt

SEQ ID NO: 45 - DNA, 22 bp, Artificial Sequence
  Forward primer EF_Forward2
tttaggcctagagaaggtggcg

SEQ ID NO: 46 - DNA, 30 bp, Artificial Sequence
  Reverse primer EF_Reverse1&2
tttaggcctgcgtaaccaccacacccgccg

SEQ ID NO: 47 - DNA, 24 bp, Artificial Sequence
  Forward primer EF_Forward3
tttaggcctttttcccgagggtgg

SEQ ID NO: 48 - DNA, 27 bp, Artificial Sequence
  Reverse primer EF_Reverse3
tttaggcctcagtgatgacgagagcgg